European Patent Specification EP 3 536 712 B1, published May 31, 2023. Title: Methods for Reducing Lipoprotein(a) Levels by Administering an Inhibitor of Proprotein Convertase Subtilisin Kexin-9 (PCSK9). Applicant: Regeneron Pharmaceuticals, Inc. Application To be assigned. The sequence listing filed with the application follows.

SEQUENCE LISTING (763 sequences)

SEQ ID NO: 1 - DNA, 351 bp, Artificial Sequence
  Synthetic
caggtccagctggtgcagtctgggggaggcttggtacagcctggggggtccctgagactctcctgtgcagcctctggatttactctaagtagttacgacatgcactgggtccgccaatctacaggaaaaggtctggagtgggtctcagctattggttctaccggtgacacatactatccaggctccgtgaagggccgattcaccatcaccagagaaaaagccaagaactccgtgtatcttcaaatgaacagcctgagagccggggacacggctgtgtattactgtgtaagagaggggtgggaggtaccctttgactactggggccagggaaccctggtcactgtctcctca

SEQ ID NO: 2 - protein, 117 aa, Artificial Sequence
  Synthetic
QVQLVQSGGGLVQPGGSLRLSCAASGFTLSSYDMHWVRQSTGKGLEWVSAIGSTGDTYYPGSVKGRFTITREKAKNSVYLQMNSLRAGDTAVYYCVREGWEVPFDYWGQGTLVTVSS

SEQ ID NO: 3 - DNA, 24 bp, Artificial Sequence
  Synthetic
ggatttactctaagtagttacgac

SEQ ID NO: 4 - protein, 8 aa, Artificial Sequence
  Synthetic
GFTLSSYD

SEQ ID NO: 5 - DNA, 21 bp, Artificial Sequence
  Synthetic
attggttctaccggtgacaca

SEQ ID NO: 6 - protein, 7 aa, Artificial Sequence
  Synthetic
IGSTGDT

SEQ ID NO: 7 - DNA, 33 bp, Artificial Sequence
  Synthetic
gtaagagaggggtgggaggtaccctttgactac

SEQ ID NO: 8 - protein, 11 aa, Artificial Sequence
  Synthetic
VREGWEVPFDY

SEQ ID NO: 9 - DNA, 327 bp, Artificial Sequence
  Synthetic
gacatccagatgacccagtctccagccaccctgtctgtgtctccaggggaaagagccgccctctcctgcagggccagtcagagtgttagcagcaacttagcctggtaccaccagaaacctggccaggctcccaggctcctcatctatggtgcatccaccagggccactggtatcccagccaggttcagtggcattgggtctgggacagagttcactctcattatcagcagcctgcagtctgaagattttgcattttatttctgtcagcagtataataactggcctccattcactttcggccctgggaccaaggtggagatcaaacga

SEQ ID NO: 10 - protein, 109 aa, Artificial Sequence
  Synthetic
DIQMTQSPATLSVSPGERAALSCRASQSVSSNLAWYHQKPGQAPRLLIYGASTRATGIPARFSGIGSGTEFTLIISSLQSEDFAFYFCQQYNNWPPFTFGPGTKVEIKR

SEQ ID NO: 11 - DNA, 18 bp, Artificial Sequence
  Synthetic
cagagtgttagcagcaac

SEQ ID NO: 12 - protein, 6 aa, Artificial Sequence
  Synthetic
QSVSSN

SEQ ID NO: 13 - DNA, 9 bp, Artificial Sequence
  Synthetic
ggtgcatcc

SEQ ID NO: 14 - protein, 3 aa, Artificial Sequence
  Synthetic
GAS

SEQ ID NO: 15 - DNA, 30 bp, Artificial Sequence
  Synthetic
cagcagtataataactggcctccattcact

SEQ ID NO: 16 - protein, 10 aa, Artificial Sequence
  Synthetic
QQYNNWPPFT

SEQ ID NO: 17 - DNA, 351 bp, Artificial Sequence
  Synthetic
gaggtgcagctggtggagtctgggggaggcttggtacagcctggggggtccctgagactctcctgtgcagcctctggatttactctaagtagttacgacatgcactgggtccgccaatctacaggaaaaggtctggagtgggtctcagctattggttctaccggtgacacatactatccaggctccgtgaagggccgattcaccatcaccagagaaaaagccaagaactccgtgtatcttcaaatgaacagcctgagagccggggacacggctgtgtattactgtgtaagagaggggtgggaggtaccctttgactactggggccagggaaccctggtcaccgtctcctca

SEQ ID NO: 18 - protein, 117 aa, Artificial Sequence
  Synthetic
EVQLVESGGGLVQPGGSLRLSCAASGFTLSSYDMHWVRQSTGKGLEWVSAIGSTGDTYYPGSVKGRFTITREKAKNSVYLQMNSLRAGDTAVYYCVREGWEVPFDYWGQGTLVTVSS

SEQ ID NO: 19 - DNA, 324 bp, Artificial Sequence
  Synthetic
gaaatagtgatgacgcagtctccagccaccctgtctgtgtctccaggggaaagagccgccctctcctgcagggccagtcagagtgttagcagcaacttagcctggtaccaccagaaacctggccaggctcccaggctcctcatctatggtgcatccaccagggccactggtatcccagccaggttcagtggcattgggtctgggacagagttcactctcattatcagcagcctgcagtctgaagattttgcattttatttctgtcagcagtataataactggcctccattcactttcggccctgggaccaaagtggatatcaaa

SEQ ID NO: 20 - protein, 108 aa, Artificial Sequence
  Synthetic
EIVMTQSPATLSVSPGERAALSCRASQSVSSNLAWYHQKPGQAPRLLIYGASTRATGIPARFSGIGSGTEFTLIISSLQSEDFAFYFCQQYNNWPPFTFGPGTKVDIK

SEQ ID NO: 21 - DNA, 351 bp, Artificial Sequence
  Synthetic
gaggtgcagctggtggagtctgggggaggcttggtacagcctggggggtccctgagactctcctgtgcagcctctggatttactctaagtagttacgacatgcactgggtccgccaagctacaggaaaaggtctggagtgggtctcagctattggttctaccggtgacacatactatccaggctccgtgaagggccgattcaccatctccagagaaaatgccaagaactccttgtatcttcaaatgaacagcctgagagccggggacacggctgtgtattactgtgtaagagaggggtgggaggtaccctttgactactggggccagggaaccctggtcaccgtctcctca

SEQ ID NO: 22 - protein, 117 aa, Artificial Sequence
  Synthetic
EVQLVESGGGLVQPGGSLRLSCAASGFTLSSYDMHWVRQATGKGLEWVSAIGSTGDTYYPGSVKGRFTISRENAKNSLYLQMNSLRAGDTAVYYCVREGWEVPFDYWGQGTLVTVSS

SEQ ID NO: 23 - DNA, 324 bp, Artificial Sequence
  Synthetic
gaaatagtgatgacgcagtctccagccaccctgtctgtgtctccaggggaaagagccaccctctcctgcagggccagtcagagtgttagcagcaacttagcctggtaccagcagaaacctggccaggctcccaggctcctcatctatggtgcatccaccagggccactggtatcccagccaggttcagtggcagtgggtctgggacagagttcactctcaccatcagcagcctgcagtctgaagattttgcagtttattactgtcagcagtataataactggcctccattcactttcggccctgggaccaaagtggatatcaaa

SEQ ID NO: 24 - protein, 108 aa, Artificial Sequence
  Synthetic
EIVMTQSPATLSVSPGERATLSCRASQSVSSNLAWYQQKPGQAPRLLIYGASTRATGIPARFSGSGSGTEFTLTISSLQSEDFAVYYCQQYNNWPPFTFGPGTKVDIK

SEQ ID NO: 25 - DNA, 342 bp, Artificial Sequence
  Synthetic
caggtgcagctggtgcagtctgggggaggcgtggtccagcctgggaggtccctgagactctcctgtgcagcgtctggattcaccttcagtagctatggcatgcactgggtccgccaggctccaggcaaggggctggagtgggtggcgtttataggatttgatggaagtaatatacattatggagactccgtgaggggccgaatcatcatatccagagacaattccgagaacacgttgtatctggaaatgaacagcctgagagccgaggacacggcaatgtactattgtgcgagagagaagggtttagactggggccagggaaccacggtcaccgtctcctca

SEQ ID NO: 26 - protein, 114 aa, Artificial Sequence
  Synthetic
QVQLVQSGGGVVQPGRSLRLSCAASGFTFSSYGMHWVRQAPGKGLEWVAFIGFDGSNIHYGDSVRGRIIISRDNSENTLYLEMNSLRAEDTAMYYCAREKGLDWGQGTTVTVSS

SEQ ID NO: 27 - DNA, 24 bp, Artificial Sequence
  Synthetic
ggattcaccttcagtagctatggc

SEQ ID NO: 28 - protein, 8 aa, Artificial Sequence
  Synthetic
GFTFSSYG

SEQ ID NO: 29 - DNA, 24 bp, Artificial Sequence
  Synthetic
ataggatttgatggaagtaatata

SEQ ID NO: 30 - protein, 8 aa, Artificial Sequence
  Synthetic
IGFDGSNI

SEQ ID NO: 31 - DNA, 21 bp, Artificial Sequence
  Synthetic
gcgagagagaagggtttagac

SEQ ID NO: 32 - protein, 7 aa, Artificial Sequence
  Synthetic
AREKGLD

SEQ ID NO: 33 - DNA, 321 bp, Artificial Sequence
  Synthetic
gccatccagatgacccagtctccttccaccctgtctgcatctgtaggagacagagtcaccatcacttgccgggccagtcagagtattagtagctggttggcctggtatcagcagaaaccagggaaagcccctaagctcctgatctataaggcgtctagtttagaaagtggggtcccatcaaggttcagcggcagtggatctgggacagaattcactctcaccatcagcagcctgcagcctgatgattttgcaacttattactgccaacagtataatagttattacacttttggccaggggaccaaggtggaaatcaaacga

SEQ ID NO: 34 - protein, 107 aa, Artificial Sequence
  Synthetic
AIQMTQSPSTLSASVGDRVTITCRASQSISSWLAWYQQKPGKAPKLLIYKASSLESGVPSRFSGSGSGTEFTLTISSLQPDDFATYYCQQYNSYYTFGQGTKVEIKR

SEQ ID NO: 35 - DNA, 18 bp, Artificial Sequence
  Synthetic
cagagtattagtagctgg

SEQ ID NO: 36 - protein, 6 aa, Artificial Sequence
  Synthetic
QSISSW

SEQ ID NO: 37 - DNA, 9 bp, Artificial Sequence
  Synthetic
aaggcgtct

SEQ ID NO: 38 - protein, 3 aa, Artificial Sequence
  Synthetic
KAS

SEQ ID NO: 39 - DNA, 24 bp, Artificial Sequence
  Synthetic
caacagtataatagttattacact

SEQ ID NO: 40 - protein, 8 aa, Artificial Sequence
  Synthetic
QQYNSYYT

SEQ ID NO: 41 - DNA, 342 bp, Artificial Sequence
  Synthetic
caggtgcagctggtggagtctgggggaggcgtggtccagcctgggaggtccctgagactctcctgtgcagcgtctggattcaccttcagtagctatggcatgcactgggtccgccaggctccaggcaaggggctggagtgggtggcgtttataggatttgatggaagtaatatacattatggagactccgtgaggggccgaatcatcatatccagagacaattccgagaacacgttgtatctggaaatgaacagcctgagagccgaggacacggcaatgtactattgtgcgagagagaagggtttagactggggccagggaaccctggtcaccgtctcctca

SEQ ID NO: 42 - protein, 114 aa, Artificial Sequence
  Synthetic
QVQLVESGGGVVQPGRSLRLSCAASGFTFSSYGMHWVRQAPGKGLEWVAFIGFDGSNIHYGDSVRGRIIISRDNSENTLYLEMNSLRAEDTAMYYCAREKGLDWGQGTLVTVSS

SEQ ID NO: 43 - DNA, 318 bp, Artificial Sequence
  Synthetic
gacatccagatgacccagtctccttccaccctgtctgcatctgtaggagacagagtcaccatcacttgccgggccagtcagagtattagtagctggttggcctggtatcagcagaaaccagggaaagcccctaagctcctgatctataaggcgtctagtttagaaagtggggtcccatcaaggttcagcggcagtggatctgggacagaattcactctcaccatcagcagcctgcagcctgatgattttgcaacttattactgccaacagtataatagttattacacttttggccaggggaccaagctggagatcaaa

SEQ ID NO: 44 - protein, 106 aa, Artificial Sequence
  Synthetic
DIQMTQSPSTLSASVGDRVTITCRASQSISSWLAWYQQKPGKAPKLLIYKASSLESGVPSRFSGSGSGTEFTLTISSLQPDDFATYYCQQYNSYYTFGQGTKLEIK

SEQ ID NO: 45 - DNA, 342 bp, Artificial Sequence
  Synthetic
caggtgcagctggtggagtctgggggaggcgtggtccagcctgggaggtccctgagactctcctgtgcagcctctggattcaccttcagtagctatggcatgcactgggtccgccaggctccaggcaaggggctggagtgggtggcagttataggatttgatggaagtaatatatactatgcagactccgtgaagggccgattcaccatctccagagacaattccaagaacacgctgtatctgcaaatgaacagcctgagagctgaggacacggctgtgtattactgtgcgagagagaagggtttagactggggccagggaaccctggtcaccgtctcctca

SEQ ID NO: 46 - protein, 114 aa, Artificial Sequence
  Synthetic
QVQLVESGGGVVQPGRSLRLSCAASGFTFSSYGMHWVRQAPGKGLEWVAVIGFDGSNIYYADSVKGRFTISRDNSKNTLYLQMNSLRAEDTAVYYCAREKGLDWGQGTLVTVSS

SEQ ID NO: 47 - DNA, 319 bp, Artificial Sequence
  Synthetic
gacatccagatgacccagtctccttccaccctgtctgcatctgtaggagacagagtcaccatcacttgccgggccagtcagagtattagtagctggttggcctggtatcagcagaaaccagggaaagcccctaagctcctgatctataaggcgtctagtttagaaagtggggtcccatcaaggttcagcggcagtggatctgggacagaattcactctcaccatcagcagcctgcagcctgatgattttgcaacttattactgccaacagtataatagttattacacttttggccaggggaccaagctggagatcaaac

SEQ ID NO: 48 - protein, 106 aa, Artificial Sequence; identical to SEQ ID NO: 44
  Synthetic

SEQ ID NO: 49 - DNA, 342 bp, Artificial Sequence
  Synthetic
caggtgcagctgcaggagtctgggggaggcgtggtccagcctgggaggtccctgagactctcctgtgcagcgtctggattcaccttcagtagctatggcatgcactgggtccgccaggctccaggcaaggggctggagtgggtggcgtttataggatttgatggaagtaatatatattatggagactccgtgaggggccgaatcatcatatccagagacaattccgagaacacgttgtatctggaaatgaacagcctgagagccgaggacacggcagtgtattattgtgcgagagagaagggtttagactggggccagggaaccctggtcactgtctcctca

SEQ ID NO: 50 - protein, 114 aa, Artificial Sequence
  Synthetic
QVQLQESGGGVVQPGRSLRLSCAASGFTFSSYGMHWVRQAPGKGLEWVAFIGFDGSNIYYGDSVRGRIIISRDNSENTLYLEMNSLRAEDTAVYYCAREKGLDWGQGTLVTVSS

SEQ ID NO: 51 - DNA, 24 bp, Artificial Sequence
  Synthetic
ggattcaccttcagtagctatggc

SEQ ID NO: 52 - protein, 8 aa, Artificial Sequence
  Synthetic
GFTFSSYG

SEQ ID NO: 53 - DNA, 24 bp, Artificial Sequence
  Synthetic
ataggatttgatggaagtaatata

SEQ ID NO: 54 - protein, 8 aa, Artificial Sequence
  Synthetic
IGFDGSNI

SEQ ID NO: 55 - DNA, 21 bp, Artificial Sequence
  Synthetic
gcgagagagaagggtttagac

SEQ ID NO: 56 - protein, 7 aa, Artificial Sequence
  Synthetic
AREKGLD

SEQ ID NO: 57 - DNA, 342 bp, Artificial Sequence
  Synthetic
gccatccagatgacccagtctccagactccctggctgtgtctctgggcgagagggccaccatcaactgcaagtccagccagagtgtttttcacacctccaacaataagaactacttagtttggtatcagcagaaaccaggacagcctcctaagttgctcctttactgggcctctacccgggaatccggggtccctgaccgattcagtggcagcgggtctgggacagatttcactctcaccatcagcagcctgcaggctgaagatgtggcaaattattactgtcaccaatattacagtattccgtggacgttcggccaagggaccaaggtggagatcaaacga

SEQ ID NO: 58 - protein, 114 aa, Artificial Sequence
  Synthetic
AIQMTQSPDSLAVSLGERATINCKSSQSVFHTSNNKNYLVWYQQKPGQPPKLLLYWASTRESGVPDRFSGSGSGTDFTLTISSLQAEDVANYYCHQYYSIPWTFGQGTKVEIKR

SEQ ID NO: 59 - DNA, 36 bp, Artificial Sequence
  Synthetic
cagagtgtttttcacacctccaacaataagaactac

SEQ ID NO: 60 - protein, 12 aa, Artificial Sequence
  Synthetic
QSVFHTSNNKNY

SEQ ID NO: 61 - DNA, 9 bp, Artificial Sequence
  Synthetic
tgggcctct

SEQ ID NO: 62 - protein, 3 aa, Artificial Sequence
  Synthetic
WAS

SEQ ID NO: 63 - DNA, 27 bp, Artificial Sequence
  Synthetic
caccaatattacagtattccgtggacg

SEQ ID NO: 64 - protein, 9 aa, Artificial Sequence
  Synthetic
HQYYSIPWT

SEQ ID NO: 65 - DNA, 342 bp, Artificial Sequence
  Synthetic
caggtgcagctggtggagtctgggggaggcgtggtccagcctgggaggtccctgagactctcctgtgcagcgtctggattcaccttcagtagctatggcatgcactgggtccgccaggctccaggcaaggggctggagtgggtggcgtttataggatttgatggaagtaatatatattatggagactccgtgaggggccgaatcatcatatccagagacaattccgagaacacgttgtatctggaaatgaacagcctgagagccgaggacacggcagtgtattattgtgcgagagagaagggtttagactggggccagggaaccctggtcaccgtctcctca

SEQ ID NO: 66 - protein, 114 aa, Artificial Sequence
  Synthetic
QVQLVESGGGVVQPGRSLRLSCAASGFTFSSYGMHWVRQAPGKGLEWVAFIGFDGSNIYYGDSVRGRIIISRDNSENTLYLEMNSLRAEDTAVYYCAREKGLDWGQGTLVTVSS

SEQ ID NO: 67 - DNA, 339 bp, Artificial Sequence
  Synthetic
gacatcgtgatgacccagtctccagactccctggctgtgtctctgggcgagagggccaccatcaactgcaagtccagccagagtgtttttcacacctccaacaataagaactacttagtttggtatcagcagaaaccaggacagcctcctaagttgctcctttactgggcctctacccgggaatccggggtccctgaccgattcagtggcagcgggtctgggacagatttcactctcaccatcagcagcctgcaggctgaagatgtggcaaattattactgtcaccaatattacagtattccgtggacgttcggccaagggaccaaggtggaaatcaaa

SEQ ID NO: 68 - protein, 113 aa, Artificial Sequence
  Synthetic
DIVMTQSPDSLAVSLGERATINCKSSQSVFHTSNNKNYLVWYQQKPGQPPKLLLYWASTRESGVPDRFSGSGSGTDFTLTISSLQAEDVANYYCHQYYSIPWTFGQGTKVEIK

SEQ ID NO: 69 - DNA, 342 bp, Artificial Sequence; identical to SEQ ID NO: 45
  Synthetic

SEQ ID NO: 70 - protein, 114 aa, Artificial Sequence; identical to SEQ ID NO: 46
  Synthetic

SEQ ID NO: 71 - DNA, 339 bp, Artificial Sequence
  Synthetic
gacatcgtgatgacccagtctccagactccctggctgtgtctctgggcgagagggccaccatcaactgcaagtccagccagagtgtttttcacacctccaacaataagaactacttagcttggtaccagcagaaaccaggacagcctcctaagctgctcatttactgggcctctacccgggaatccggggtccctgaccgattcagtggcagcgggtctgggacagatttcactctcaccatcagcagcctgcaggctgaagatgtggcagtttattactgtcaccaatattacagtattccgtggacgttcggccaagggaccaaggtggaaatcaaa

SEQ ID NO: 72 - protein, 113 aa, Artificial Sequence
  Synthetic
DIVMTQSPDSLAVSLGERATINCKSSQSVFHTSNNKNYLAWYQQKPGQPPKLLIYWASTRESGVPDRFSGSGSGTDFTLTISSLQAEDVAVYYCHQYYSIPWTFGQGTKVEIK

SEQ ID NO: 73 - DNA, 354 bp, Artificial Sequence
  Synthetic
gaagtgcagctggtgcagtctgggggaggcttggtacagcctggggggtccctgagactctcctgtgcagcctctggattcacctttaacaactatgccatgaactgggtccgccaggctccaggaaagggactggactgggtctcaactattagtggtagcggtggtactacaaactacgcagactccgtgaagggccgtttcattatttcccgagacagttccaaacacacgctgtatctgcaaatgaacagcctgagagccgaggacacggccgtatattactgtgcgaaagattctaactggggaaatttcgatctctggggccgtggcaccacggtcactgtctcctca

SEQ ID NO: 74 - protein, 118 aa, Artificial Sequence
  Synthetic
EVQLVQSGGGLVQPGGSLRLSCAASGFTFNNYAMNWVRQAPGKGLDWVSTISGSGGTTNYADSVKGRFIISRDSSKHTLYLQMNSLRAEDTAVYYCAKDSNWGNFDLWGRGTTVTVSS

SEQ ID NO: 75 - DNA, 24 bp, Artificial Sequence
  Synthetic
ggattcacctttaacaactatgcc

SEQ ID NO: 76 - protein, 8 aa, Artificial Sequence
  Synthetic
GFTFNNYA

SEQ ID NO: 77 - DNA, 24 bp, Artificial Sequence
  Synthetic
attagtggtagcggtggtactaca

SEQ ID NO: 78 - protein, 8 aa, Artificial Sequence
  Synthetic
ISGSGGTT

SEQ ID NO: 79 - DNA, 33 bp, Artificial Sequence
  Synthetic
gcgaaagattctaactggggaaatttcgatctc

SEQ ID NO: 80 - protein, 11 aa, Artificial Sequence
  Synthetic
AKDSNWGNFDL

SEQ ID NO: 81 - DNA, 342 bp, Artificial Sequence
  Synthetic
gacatccagatgacccagtctccagactccctggctgtgtctctgggcgagagggccaccatcaactgcaagtccagccagagtgttttatacaggtccaacaataggaacttcttaggttggtaccagcagaaaccagggcagcctcctaatctactcatttactgggcatctacccgggaatccggggtccctgaccgattcagtggcagcgggtctgggacagatttcactctcaccatcagcagcctgcaggctgaagatgtggcagtttattactgtcaacaatattatactactccgtacacttttggccaggggaccaaggtggaaatcaaacga

SEQ ID NO: 82 - protein, 114 aa, Artificial Sequence
  Synthetic
DIQMTQSPDSLAVSLGERATINCKSSQSVLYRSNNRNFLGWYQQKPGQPPNLLIYWASTRESGVPDRFSGSGSGTDFTLTISSLQAEDVAVYYCQQYYTTPYTFGQGTKVEIKR

SEQ ID NO: 83 - DNA, 36 bp, Artificial Sequence
  Synthetic
cagagtgttttatacaggtccaacaataggaacttc

SEQ ID NO: 84 - protein, 12 aa, Artificial Sequence
  Synthetic
QSVLYRSNNRNF

SEQ ID NO: 85 - DNA, 9 bp, Artificial Sequence
  Synthetic
tgggcatct

SEQ ID NO: 86 - protein, 3 aa, Artificial Sequence
  Synthetic
WAS

SEQ ID NO: 87 - DNA, 27 bp, Artificial Sequence
  Synthetic
caacaatattatactactccgtacact

SEQ ID NO: 88 - protein, 9 aa, Artificial Sequence
  Synthetic
QQYYTTPYT

SEQ ID NO: 89 - DNA, 354 bp, Artificial Sequence
  Synthetic
gaggtgcagctggtggagtctgggggaggcttggtacagcctggggggtccctgagactctcctgtgcagcctctggattcacctttaacaactatgccatgaactgggtccgccaggctccaggaaagggactggactgggtctcaactattagtggtagcggtggtactacaaactacgcagactccgtgaagggccgtttcattatttcccgagacagttccaaacacacgctgtatctgcaaatgaacagcctgagagccgaggacacggccgtatattactgtgcgaaagattctaactggggaaatttcgatctctggggccgtggcaccctggtcactgtctcctca

SEQ ID NO: 90 - protein, 118 aa, Artificial Sequence [sequence omitted]

SEQ ID NO: 91 - DNA, 339 bp, Artificial Sequence
  Synthetic
gacatcgtgatgacccagtctccagactccctggctgtgtctctgggcgagagggccaccatcaactgcaagtccagccagagtgttttatacaggtccaacaataggaacttcttaggttggtaccagcagaaaccagggcagcctcctaatctactcatttactgggcatctacccgggaatccggggtccctgaccgattcagtggcagcgggtctgggacagatttcactctcaccatcagcagcctgcaggctgaagatgtggcagtttattactgtcaacaatattatactactccgtacacttttggccaggggaccaagctggagatcaaa

SEQ ID NO: 92 - protein, 113 aa, Artificial Sequence [sequence omitted]

SEQ ID NO: 93 - DNA, 354 bp, Artificial Sequence
  Synthetic
gaggtgcagctggtggagtctgggggaggcttggtacagcctggggggtccctgagactctcctgtgcagcctctggattcacctttaacaactatgccatgagctgggtccgccaggctccagggaaggggctggagtgggtctcagctattagtggtagcggtggtactacatactacgcagactccgtgaagggccggttcaccatctccagagacaattccaagaacacgctgtatctgcaaatgaacagcctgagagccgaggacacggccgtatattactgtgcgaaagattctaactggggaaatttcgatctctggggccgtggcaccctggtcactgtctcctca

SEQ ID NO: 94 - protein, 118 aa, Artificial Sequence
  Synthetic
EVQLVESGGGLVQPGGSLRLSCAASGFTFNNYAMSWVRQAPGKGLEWVSAISGSGGTTYYADSVKGRFTISRDNSKNTLYLQMNSLRAEDTAVYYCAKDSNWGNFDLWGRGTLVTVSS

SEQ ID NO: 95 - DNA, 339 bp, Artificial Sequence
  Synthetic
gacatcgtgatgacccagtctccagactccctggctgtgtctctgggcgagagggccaccatcaactgcaagtccagccagagtgttttatacaggtccaacaataggaacttcttagcttggtaccagcagaaaccaggacagcctcctaagctgctcatttactgggcatctacccgggaatccggggtccctgaccgattcagtggcagcgggtctgggacagatttcactctcaccatcagcagcctgcaggctgaagatgtggcagtttattactgtcaacaatattatactactccgtacacttttggccaggggaccaagctggagatcaaa

SEQ ID NO: 96 - protein, 113 aa, Artificial Sequence
  Synthetic
DIVMTQSPDSLAVSLGERATINCKSSQSVLYRSNNRNFLAWYQQKPGQPPKLLIYWASTRESGVPDRFSGSGSGTDFTLTISSLQAEDVAVYYCQQYYTTPYTFGQGTKLEIK

SEQ ID NO: 97 - DNA, 351 bp, Artificial Sequence
  Synthetic
caggtgcagctggtgcagtctgggggaggcttggtacagcctggggggtccctgagactctcctgtgcagtctctggattcaccctcagtagctacgatatgcactgggtccgccaacctacaggaaaaggtctggagtgggtctcagctattggttctactggtgacacatactatccaggctccgtgaagggccgattcaccatctccagagaaaatgccaagaactccttgtatcttcaaatgaacagcctgagagccggggacacggctgtgtattactgtgcaagagagggatgggacgtaccctttgacttctggggccagggaaccctggtcaccgtctcctca

SEQ ID NO: 98 - protein, 117 aa, Artificial Sequence
  Synthetic
QVQLVQSGGGLVQPGGSLRLSCAVSGFTLSSYDMHWVRQPTGKGLEWVSAIGSTGDTYYPGSVKGRFTISRENAKNSLYLQMNSLRAGDTAVYYCAREGWDVPFDFWGQGTLVTVSS

SEQ ID NO: 99 - DNA, 24 bp, Artificial Sequence
  Synthetic
ggattcaccctcagtagctacgat

SEQ ID NO: 100 - protein, 8 aa, Artificial Sequence
  Synthetic
GFTLSSYD

SEQ ID NO: 101 - DNA, 21 bp, Artificial Sequence
  Synthetic
attggttctactggtgacaca

SEQ ID NO: 102 - protein, 7 aa, Artificial Sequence
  Synthetic
IGSTGDT

SEQ ID NO: 103 - DNA, 33 bp, Artificial Sequence
  Synthetic
gcaagagagggatgggacgtaccctttgacttc

SEQ ID NO: 104 - protein, 11 aa, Artificial Sequence
  Synthetic
AREGWDVPFDF

SEQ ID NO: 105 - DNA, 324 bp, Artificial Sequence
  Synthetic
gccatccagttgacccagtctccatcctccctgtctgcatctgtaggagacagagtcaccatcacttgccgggcaagtcaggacattagaaatgatttaggctggtatcagcagaaaccagggaaagcccctaagctcctgatctatgctgcatccagtttacaaagtggggtcccatcacggttcagcggcagtggatctggcacagatttcactctcaccatcagcagcctgcagcctgaagattttgcaacttattactgtctacaagattacaattacccgtggacgttcggccaagggaccaaggtggagatcaaacga

SEQ ID NO: 106 - protein, 108 aa, Artificial Sequence
  Synthetic
AIQLTQSPSSLSASVGDRVTITCRASQDIRNDLGWYQQKPGKAPKLLIYAASSLQSGVPSRFSGSGSGTDFTLTISSLQPEDFATYYCLQDYNYPWTFGQGTKVEIKR

SEQ ID NO: 107 - DNA, 18 bp, Artificial Sequence
  Synthetic
caggacattagaaatgat

SEQ ID NO: 108 - protein, 6 aa, Artificial Sequence
  Synthetic
QDIRND

SEQ ID NO: 109 - DNA, 9 bp, Artificial Sequence
  Synthetic
gctgcatcc

SEQ ID NO: 110 - protein, 3 aa, Artificial Sequence
  Synthetic
AAS

SEQ ID NO: 111 - DNA, 27 bp, Artificial Sequence
  Synthetic
ctacaagattacaattacccgtggacg

SEQ ID NO: 112 - protein, 9 aa, Artificial Sequence
  Synthetic
LQDYNYPWT

SEQ ID NO: 113 - DNA, 351 bp, Artificial Sequence
  Synthetic
gaggtgcagctggtggagtctgggggaggcttggtacagcctggggggtccctgagactctcctgtgcagtctctggattcaccctcagtagctacgatatgcactgggtccgccaacctacaggaaaaggtctggagtgggtctcagctattggttctactggtgacacatactatccaggctccgtgaagggccgattcaccatctccagagaaaatgccaagaactccttgtatcttcaaatgaacagcctgagagccggggacacggctgtgtattactgtgcaagagagggatgggacgtaccctttgacttctggggccagggaaccctggtcaccgtctcctca

SEQ ID NO: 114 - protein, 117 aa, Artificial Sequence
  Synthetic
EVQLVESGGGLVQPGGSLRLSCAVSGFTLSSYDMHWVRQPTGKGLEWVSAIGSTGDTYYPGSVKGRFTISRENAKNSLYLQMNSLRAGDTAVYYCAREGWDVPFDFWGQGTLVTVSS

SEQ ID NO: 115 - DNA, 321 bp, Artificial Sequence
  Synthetic
gccatccagatgacccagtctccatcctccctgtctgcatctgtaggagacagagtcaccatcacttgccgggcaagtcaggacattagaaatgatttaggctggtatcagcagaaaccagggaaagcccctaagctcctgatctatgctgcatccagtttacaaagtggggtcccatcacggttcagcggcagtggatctggcacagatttcactctcaccatcagcagcctgcagcctgaagattttgcaacttattactgtctacaagattacaattacccgtggacgttcggccaagggaccaaggtggaaatcaaa

SEQ ID NO: 116 - protein, 107 aa, Artificial Sequence
  Synthetic
AIQMTQSPSSLSASVGDRVTITCRASQDIRNDLGWYQQKPGKAPKLLIYAASSLQSGVPSRFSGSGSGTDFTLTISSLQPEDFATYYCLQDYNYPWTFGQGTKVEIK

SEQ ID NO: 117 - DNA, 351 bp, Artificial Sequence
  Synthetic
gaggtgcagctggtggagtctgggggaggcttggtacagcctggggggtccctgagactctcctgtgcagcctctggattcaccctcagtagctacgatatgcactgggtccgccaagctacaggaaaaggtctggagtgggtctcagctattggttctactggtgacacatactatccaggctccgtgaagggccgattcaccatctccagagaaaatgccaagaactccttgtatcttcaaatgaacagcctgagagccggggacacggctgtgtattactgtgcaagagagggatgggacgtaccctttgacttctggggccagggaaccctggtcaccgtctcctca

SEQ ID NO: 118 - protein, 117 aa, Artificial Sequence
  Synthetic
EVQLVESGGGLVQPGGSLRLSCAASGFTLSSYDMHWVRQATGKGLEWVSAIGSTGDTYYPGSVKGRFTISRENAKNSLYLQMNSLRAGDTAVYYCAREGWDVPFDFWGQGTLVTVSS

SEQ ID NO: 119 - DNA, 321 bp, Artificial Sequence
  Synthetic
gccatccagatgacccagtctccatcctccctgtctgcatctgtaggagacagagtcaccatcacttgccgggcaagtcaggacattagaaatgatttaggctggtatcagcagaaaccagggaaagcccctaagctcctgatctatgctgcatccagtttacaaagtggggtcccatcaaggttcagcggcagtggatctggcacagatttcactctcaccatcagcagcctgcagcctgaagattttgcaacttattactgtctacaagattacaattacccgtggacgttcggccaagggaccaaggtggaaatcaaa

SEQ ID NO: 120 - protein, 107 aa, Artificial Sequence; identical to SEQ ID NO: 116
  Synthetic

SEQ ID NO: 121 - DNA, 384 bp, Artificial Sequence
  Synthetic
caggtgcagctgcaggagtcggggccaggactggtgaagccttcggagaccctgtccctcacctgcactgtctctggggactccatcaatacttactactggagctggttccggcagcccccagggaagggactggagtggattgggtatatctattatagtggaaccaccaactacaacccctccctcaagagtcgagtcaccatatcaatagacacgcccaggaaccagttctccctgaagctgatctctgtgaccgcagcggacacggccgtgtattactgtgcgagagagaggattactatgattcggggagttaccctctactattactcctacggtatggacgtctggggccaagggaccacggtcaccgtctcctca

SEQ ID NO: 122 - protein, 128 aa, Artificial Sequence
  Synthetic
QVQLQESGPGLVKPSETLSLTCTVSGDSINTYYWSWFRQPPGKGLEWIGYIYYSGTTNYNPSLKSRVTISIDTPRNQFSLKLISVTAADTAVYYCARERITMIRGVTLYYYSYGMDVWGQGTTVTVSS

SEQ ID NO: 123 - DNA, 24 bp, Artificial Sequence
  Synthetic
ggggactccatcaatacttactac

SEQ ID NO: 124 - protein, 8 aa, Artificial Sequence
  Synthetic
GDSINTYY

SEQ ID NO: 125 - DNA, 21 bp, Artificial Sequence
  Synthetic
atctattatagtggaaccacc

SEQ ID NO: 126 - protein, 7 aa, Artificial Sequence
  Synthetic
IYYSGTT

SEQ ID NO: 127 - DNA, 66 bp, Artificial Sequence
  Synthetic
gcgagagagaggattactatgattcggggagttaccctctactattactcctacggtatggacgtc

SEQ ID NO: 128 - protein, 22 aa, Artificial Sequence
  Synthetic
ARERITMIRGVTLYYYSYGMDV

SEQ ID NO: 129 - DNA, 324 bp, Artificial Sequence
  Synthetic
gacatccagatgacccagtctccatccttcctgtctgcatctgtaggagacagagtcaccatcacttgctgggccagtcaggacattagcagttatttagcctggtatcagcaaaaaccagggatagcccctaagctcctgatctatgctgcatccactttgcaaagtggggtcccatcaaggttcggcggcagtggatctgggacagaattcactctcacaatcagcagcctgcagcctgaagattttgcaacttattactgtcaacagcttaatagttaccctcggacgttcggccaagggaccaaggtggaaatcaaacga

SEQ ID NO: 130 - protein, 108 aa, Artificial Sequence
  Synthetic
DIQMTQSPSFLSASVGDRVTITCWASQDISSYLAWYQQKPGIAPKLLIYAASTLQSGVPSRFGGSGSGTEFTLTISSLQPEDFATYYCQQLNSYPRTFGQGTKVEIKR

SEQ ID NO: 131 - DNA, 18 bp, Artificial Sequence
  Synthetic
caggacattagcagttat

SEQ ID NO: 132 - protein, 6 aa, Artificial Sequence
  Synthetic
QDISSY

SEQ ID NO: 133 - DNA, 9 bp, Artificial Sequence
  Synthetic
gctgcatcc

SEQ ID NO: 134 - protein, 3 aa, Artificial Sequence
  Synthetic
AAS

SEQ ID NO: 135 - DNA, 27 bp, Artificial Sequence
  Synthetic
caacagcttaatagttaccctcggacg

SEQ ID NO: 136 - protein, 9 aa, Artificial Sequence
  Synthetic
QQLNSYPRT

SEQ ID NO: 137 - DNA, 384 bp, Artificial Sequence; identical to SEQ ID NO: 121
  Synthetic

SEQ ID NO: 138 - protein, 128 aa, Artificial Sequence; identical to SEQ ID NO: 122
  Synthetic

SEQ ID NO: 139 - DNA, 321 bp, Artificial Sequence
  Synthetic
gacatccagatgacccagtctccatccttcctgtctgcatctgtaggagacagagtcaccatcacttgctgggccagtcaggacattagcagttatttagcctggtatcagcaaaaaccagggatagcccctaagctcctgatctatgctgcatccactttgcaaagtggggtcccatcaaggttcggcggcagtggatctgggacagaattcactctcacaatcagcagcctgcagcctgaagattttgcaacttattactgtcaacagcttaatagttaccctcggacgttcggccaagggaccaaggtggaaatcaaa

SEQ ID NO: 140 - protein, 107 aa, Artificial Sequence
  Synthetic
DIQMTQSPSFLSASVGDRVTITCWASQDISSYLAWYQQKPGIAPKLLIYAASTLQSGVPSRFGGSGSGTEFTLTISSLQPEDFATYYCQQLNSYPRTFGQGTKVEIK

SEQ ID NO: 141 - DNA, 384 bp, Artificial Sequence
  Synthetic
caggtgcagctgcaggagtcgggcccaggactggtgaagccttcggagaccctgtccctcacctgcactgtctctggggactccatcaatacttactactggagctggatccggcagcccccagggaagggactggagtggattgggtatatctattatagtggaaccaccaactacaacccctccctcaagagtcgagtcaccatatcagtagacacgtccaagaaccagttctccctgaagctgagctctgtgaccgctgcggacacggccgtgtattactgtgcgagagagaggattactatgattcggggagttaccctctactattactcctacggtatggacgtctggggccaagggaccacggtcaccgtctcctca

SEQ ID NO: 142 - protein, 128 aa, Artificial Sequence
  Synthetic
QVQLQESGPGLVKPSETLSLTCTVSGDSINTYYWSWIRQPPGKGLEWIGYIYYSGTTNYNPSLKSRVTISVDTSKNQFSLKLSSVTAADTAVYYCARERITMIRGVTLYYYSYGMDVWGQGTTVTVSS

SEQ ID NO: 143 - DNA, 321 bp, Artificial Sequence
  Synthetic
gacatccagatgacccagtctccatcctccctgtctgcatctgtaggagacagagtcaccatcacttgccgggcaagtcaggacattagcagttatttaggctggtatcagcagaaaccagggaaagcccctaagcgcctgatctatgctgcatccagtttgcaaagtggggtcccatcaaggttcagcggcagtggatctgggacagaattcactctcacaatcagcagcctgcagcctgaagattttgcaacttattactgtcaacagcttaatagttaccctcggacgttcggccaagggaccaaggtggaaatcaaa

SEQ ID NO: 144 - protein, 107 aa, Artificial Sequence
  Synthetic
DIQMTQSPSSLSASVGDRVTITCRASQDISSYLGWYQQKPGKAPKRLIYAASSLQSGVPSRFSGSGSGTEFTLTISSLQPEDFATYYCQQLNSYPRTFGQGTKVEIK

SEQ ID NO: 145 - DNA, 378 bp, Artificial Sequence
  Synthetic
caggtgcagctggtgcagtctggagctgaggtgaagaagcctggggcctcagtgaaggtctcctgcaaggcttctggttacacctttaccaactatggtatcagctgggtgcgacaggcccctggacaaggacttgagttaatgggatggattagtggttacaatggtaacacaaactatgcacaagaactccaggccagagtcaccatgaccacagacacatccacgagcacagcctacatggagctgaggaacctgagatctgacgacacggccgtatattactgtgcgagagatagagtcgttgtagcagctgctaattactacttttattctatggacgtctggggccaagggaccacggtcaccgtctcctca

SEQ ID NO: 146 - protein, 126 aa, Artificial Sequence
  Synthetic
QVQLVQSGAEVKKPGASVKVSCKASGYTFTNYGISWVRQAPGQGLELMGWISGYNGNTNYAQELQARVTMTTDTSTSTAYMELRNLRSDDTAVYYCARDRVVVAAANYYFYSMDVWGQGTTVTVSS

SEQ ID NO: 147 - DNA, 24 bp, Artificial Sequence
  Synthetic
ggttacacctttaccaactatggt

SEQ ID NO: 148 - protein, 8 aa, Artificial Sequence
  Synthetic
GYTFTNYG

SEQ ID NO: 149 - DNA, 24 bp, Artificial Sequence
  Synthetic
attagtggttacaatggtaacaca

SEQ ID NO: 150 - protein, 8 aa, Artificial Sequence
  Synthetic
ISGYNGNT

SEQ ID NO: 151 - DNA, 57 bp, Artificial Sequence
  Synthetic
gcgagagatagagtcgttgtagcagctgctaattactacttttattctatggacgtc

SEQ ID NO: 152 - protein, 19 aa, Artificial Sequence
  Synthetic
ARDRVVVAAANYYFYSMDV

SEQ ID NO: 153 - DNA, 339 bp, Artificial Sequence
  Synthetic
gccatccagatgacccagtctccactctccctgtccgtcacccttggacagccggcctccatctcctgcaggtctagtcaaagcctcgtatacagtgatggagacacctacttgaattggtttcagcagaggccaggccaatctccaaggcgcctaatttataaggtttctaaccgggactctggggtcccagacagattcagcggcagtgggtcaggcactgctttcacactgaaaatcagcggggtggaggccgaggatgttggggtttactactgcatgcaagctacacactggcctcggacgttcggccaagggaccaaggtggaaatcaaacga

SEQ ID NO: 154 - protein, 113 aa, Artificial Sequence
  Synthetic
AIQMTQSPLSLSVTLGQPASISCRSSQSLVYSDGDTYLNWFQQRPGQSPRRLIYKVSNRDSGVPDRFSGSGSGTAFTLKISGVEAEDVGVYYCMQATHWPRTFGQGTKVEIKR

SEQ ID NO: 155 - DNA, 33 bp, Artificial Sequence
  Synthetic
caaagcctcgtatacagtgatggagacacctac

SEQ ID NO: 156 - protein, 11 aa, Artificial Sequence
  Synthetic
QSLVYSDGDTY

SEQ ID NO: 157 - DNA, 9 bp, Artificial Sequence
  Synthetic
aaggtttct

SEQ ID NO: 158 - protein, 3 aa, Artificial Sequence
  Synthetic
KVS

SEQ ID NO: 159 - DNA, 27 bp, Artificial Sequence
  Synthetic
atgcaagctacacactggcctcggacg

SEQ ID NO: 160 - protein, 9 aa, Artificial Sequence
  Synthetic
MQATHWPRT

SEQ ID NO: 161 - DNA, 378 bp, Artificial Sequence
  Synthetic
caggttcagctggtgcagtctggagctgaggtgaagaagcctggggcctcagtgaaggtctcctgcaaggcttctggttacacctttaccaactatggtatcagctgggtgcgacaggcccctggacaaggacttgagttaatgggatggattagtggttacaatggtaacacaaactatgcacaagaactccaggccagagtcaccatgaccacagacacatccacgagcacagcctacatggagctgaggaacctgagatctgacgacacggccgtatattactgtgcgagagatagagtcgttgtagcagctgctaattactacttttattctatggacgtctggggccaagggaccacggtcaccgtctcctca

SEQ ID NO: 162 - protein, 126 aa, Artificial Sequence; identical to SEQ ID NO: 146
  Synthetic

SEQ ID NO: 163 - DNA, 336 bp, Artificial Sequence
  Synthetic
gatgttgtgatgactcagtctccactctccctgtccgtcacccttggacagccggcctccatctcctgcaggtctagtcaaagcctcgtatacagtgatggagacacctacttgaattggtttcagcagaggccaggccaatctccaaggcgcctaatttataaggtttctaaccgggactctggggtcccagacagattcagcggcagtgggtcaggcactgctttcacactgaaaatcagcggggtggaggccgaggatgttggggtttactactgcatgcaagctacacactggcctcggacgttcggccaagggaccaaggtggaaatcaaa

SEQ ID NO: 164 - protein, 112 aa, Artificial Sequence
  Synthetic
DVVMTQSPLSLSVTLGQPASISCRSSQSLVYSDGDTYLNWFQQRPGQSPRRLIYKVSNRDSGVPDRFSGSGSGTAFTLKISGVEAEDVGVYYCMQATHWPRTFGQGTKVEIK

SEQ ID NO: 165 - DNA, 378 bp, Artificial Sequence
  Synthetic
caggttcagctggtgcagtctggagctgaggtgaagaagcctggggcctcagtgaaggtctcctgcaaggcttctggttacacctttaccaactatggtatcagctgggtgcgacaggcccctggacaagggcttgagtggatgggatggattagtggttacaatggtaacacaaactatgcacagaagctccagggcagagtcaccatgaccacagacacatccacgagcacagcctacatggagctgaggagcctgagatctgacgacacggccgtgtattactgtgcgagagatagagtcgttgtagcagctgctaattactacttttattctatggacgtctggggccaagggaccacggtcaccgtctcctca

SEQ ID NO: 166 - protein, 126 aa, Artificial Sequence
  Synthetic
QVQLVQSGAEVKKPGASVKVSCKASGYTFTNYGISWVRQAPGQGLEWMGWISGYNGNTNYAQKLQGRVTMTTDTSTSTAYMELRSLRSDDTAVYYCARDRVVVAAANYYFYSMDVWGQGTTVTVSS

SEQ ID NO: 167 - DNA, 336 bp, Artificial Sequence
  Synthetic
gatgttgtgatgactcagtctccactctccctgcccgtcacccttggacagccggcctccatctcctgcaggtctagtcaaagcctcgtatacagtgatggagacacctacttgaattggtttcagcagaggccaggccaatctccaaggcgcctaatttataaggtttctaaccgggactctggggtcccagacagattcagcggcagtgggtcaggcactgatttcacactgaaaatcagcagggtggaggctgaggatgttggggtttattactgcatgcaagctacacactggcctcggacgttcggccaagggaccaaggtggaaatcaaa

SEQ ID NO: 168 - protein, 112 aa, Artificial Sequence
  Synthetic
DVVMTQSPLSLPVTLGQPASISCRSSQSLVYSDGDTYLNWFQQRPGQSPRRLIYKVSNRDSGVPDRFSGSGSGTDFTLKISRVEAEDVGVYYCMQATHWPRTFGQGTKVEIK

SEQ ID NO: 169 - DNA, 375 bp, Artificial Sequence
  Synthetic
caggtccacttgaaggagtctggtcctacgctggtgaaacccacacagaccctcacgctgacctgcaccttctctggattctcactcatcactagtggagtgggtgtgggctggattcgtcagccccccggaaaggccctggagtggcttgcactcatttattggaatggtgataagcgctacagcccatctctgaagagcaggctcaccatcaccaaggacacctccaaaaaccaggtggtccttacaatgaccaacatggaccctgtggacacagccacatattactgtgcacacaggataactgaaactagttactacttctactacggtatggacgtctggggccaagggaccacggtcaccgtctcctca

SEQ ID NO: 170 - protein, 125 aa, Artificial Sequence
  Synthetic
QVHLKESGPTLVKPTQTLTLTCTFSGFSLITSGVGVGWIRQPPGKALEWLALIYWNGDKRYSPSLKSRLTITKDTSKNQVVLTMTNMDPVDTATYYCAHRITETSYYFYYGMDVWGQGTTVTVSS

SEQ ID NO: 171 - DNA, 30 bp, Artificial Sequence
  Synthetic
ggattctcactcatcactagtggagtgggt

SEQ ID NO: 172 - protein, 10 aa, Artificial Sequence
  Synthetic
GFSLITSGVG

SEQ ID NO: 173 - DNA, 21 bp, Artificial Sequence
  Synthetic
atttattggaatggtgataag

SEQ ID NO: 174 - protein, 7 aa, Artificial Sequence
  Synthetic
IYWNGDK

SEQ ID NO: 175 - DNA, 51 bp, Artificial Sequence
  Synthetic
gcacacaggataactgaaactagttactacttctactacggtatggacgtc

SEQ ID NO: 176 - protein, 17 aa, Artificial Sequence
  Synthetic
AHRITETSYYFYYGMDV

SEQ ID NO: 177 - DNA, 339 bp, Artificial Sequence
  Synthetic
gacatccagatgacccagtctccactctccctgcccgtcacccctggagagccggcctccatctcctgcaggtctagtcagagcctcctgcatagtcatggatacgactatttggattggtacctgcagaagccagggcagtctccacagctcctgatctatttgggttctaatcgggcctccggggtccctgacaggttcagtggcagtggatcaggcacagattttacactgaaaatcagcagagtggaggctgaggatgttggggtttattactgcatgcaagctctacaaactccgctcactttcggcggagggaccaaggtggaaatcaaacga

SEQ ID NO: 178 - protein, 113 aa, Artificial Sequence
  Synthetic
DIQMTQSPLSLPVTPGEPASISCRSSQSLLHSHGYDYLDWYLQKPGQSPQLLIYLGSNRASGVPDRFSGSGSGTDFTLKISRVEAEDVGVYYCMQALQTPLTFGGGTKVEIKR

SEQ ID NO: 179 - DNA, 33 bp, Artificial Sequence
  Synthetic
cagagcctcctgcatagtcatggatacgactat

SEQ ID NO: 180 - protein, 11 aa, Artificial Sequence
  Synthetic
QSLLHSHGYDY

SEQ ID NO: 181 - DNA, 9 bp, Artificial Sequence
  Synthetic
ttgggttct

SEQ ID NO: 182 - protein, 3 aa, Artificial Sequence
  Synthetic
LGS

SEQ ID NO: 183 - DNA, 27 bp, Artificial Sequence
  Synthetic
atgcaagctctacaaactccgctcact

SEQ ID NO: 184 - protein, 9 aa, Artificial Sequence
  Synthetic
MQALQTPLT

SEQ ID NO: 185 - DNA, 375 bp, Artificial Sequence
  Synthetic
cagatcaccttgaaggagtctggtcctacgctggtgaaacccacacagaccctcacgctgacctgcaccttctctggattctcactcatcactagtggagtgggtgtgggctggattcgtcagccccccggaaaggccctggagtggcttgcactcatttattggaatggtgataagcgctacagcccatctctgaagagcaggctcaccatcaccaaggacacctccaaaaaccaggtggtccttacaatgaccaacatggaccctgtggacacagccacatattactgtgcacacaggataactgaaactagttactacttctactacggtatggacgtctggggccaagggaccacggtcaccgtctcctca

SEQ ID NO: 186 - protein, 125 aa, Artificial Sequence
  Synthetic
QITLKESGPTLVKPTQTLTLTCTFSGFSLITSGVGVGWIRQPPGKALEWLALIYWNGDKRYSPSLKSRLTITKDTSKNQVVLTMTNMDPVDTATYYCAHRITETSYYFYYGMDVWGQGTTVTVSS

SEQ ID NO: 187 - DNA, 336 bp, Artificial Sequence
  Synthetic
gatattgtgatgactcagtctccactctccctgcccgtcacccctggagagccggcctccatctcctgcaggtctagtcagagcctcctgcatagtcatggatacgactatttggattggtacctgcagaagccagggcagtctccacagctcctgatctatttgggttctaatcgggcctccggggtccctgacaggttcagtggcagtggatcaggcacagattttacactgaaaatcagcagagtggaggctgaggatgttggggtttattactgcatgcaagctctacaaactccgctcactttcggcggagggaccaaggtggagatcaaa

SEQ ID NO: 188 - protein, 112 aa, Artificial Sequence
  Synthetic
DIVMTQSPLSLPVTPGEPASISCRSSQSLLHSHGYDYLDWYLQKPGQSPQLLIYLGSNRASGVPDRFSGSGSGTDFTLKISRVEAEDVGVYYCMQALQTPLTFGGGTKVEIK

SEQ ID NO: 189 - DNA, 375 bp, Artificial Sequence
  Synthetic
cagatcaccttgaaggagtctggtcctacgctggtgaaacccacacagaccctcacgctgacctgcaccttctctggattctcactcatcactagtggagtgggtgtgggctggatccgtcagcccccaggaaaggccctggagtggcttgcactcatttattggaatggtgataagcgctacagcccatctctgaagagcaggctcaccatcaccaaggacacctccaaaaaccaggtggtccttacaatgaccaacatggaccctgtggacacagccacatattactgtgcacacaggataactgaaactagttactacttctactacggtatggacgtctggggccaagggaccacggtcaccgtctcctca

SEQ ID NO: 190 - protein, 125 aa, Artificial Sequence; identical to SEQ ID NO: 186
  Synthetic

SEQ ID NO: 191 - DNA, 336 bp, Artificial Sequence; identical to SEQ ID NO: 187
  Synthetic

SEQ ID NO: 192 - protein, 112 aa, Artificial Sequence; identical to SEQ ID NO: 188
  Synthetic

SEQ ID NO: 193 - DNA, 375 bp, Artificial Sequence
  Synthetic
cagatcaccttgaaggagtctggtcctactctggtgaaaccctcacagaccctcacgctgacctgcaccttctctgggttctcactcagcactagtggagtgggtgtgggctggatccgtcagcccccaggaaaggccctggagtggcttgcactcatttattggaattctgataagcgctacagcccatctctgaagagcaggctcaccatcaccaaggacacctccaaaaaccaggtagtccttacaatgaccaacatggaccctgtggacacagccacatattactgtgcacacagacatgacagctcgtcctactacttctactacggtatggacgtctggggccaagggatcacggtcaccgtctcctca

SEQ ID NO: 194 - protein, 125 aa, Artificial Sequence
  Synthetic
QITLKESGPTLVKPSQTLTLTCTFSGFSLSTSGVGVGWIRQPPGKALEWLALIYWNSDKRYSPSLKSRLTITKDTSKNQVVLTMTNMDPVDTATYYCAHRHDSSSYYFYYGMDVWGQGITVTVSS

SEQ ID NO: 195 - DNA, 30 bp, Artificial Sequence
  Synthetic
gggttctcactcagcactagtggagtgggt

SEQ ID NO: 196 - protein, 10 aa, Artificial Sequence
  Synthetic
GFSLSTSGVG

SEQ ID NO: 197 - DNA, 21 bp, Artificial Sequence
  Synthetic
atttattggaattctgataag

SEQ ID NO: 198 - protein, 7 aa, Artificial Sequence
  Synthetic
IYWNSDK

SEQ ID NO: 199 - DNA, 51 bp, Artificial Sequence
  Synthetic
gcacacagacatgacagctcgtcctactacttctactacggtatggacgtc

SEQ ID NO: 200 - protein, 17 aa, Artificial Sequence
  Synthetic
AHRHDSSSYYFYYGMDV

SEQ ID NO: 201 - DNA, 339 bp, Artificial Sequence
  Synthetic
gacatccagatgacccagtctccgctctccctgcccgtcacccctggagagccggcctccatctcctgcaggtctagtcagagcctcctccatagtcatggatacaactatttggattggtacctgcagaagccagggcagtctccacaactcctgatctatttgggttctaatcgggcctccggggtccctgacaggttcagtggcggtggatcaggcacagattttacactgaaaatcagcagagtggaggctgaggatgttgggatttattactgcatgcaagctctacagactcctctcactttcggcggagggaccaaggtggagatcaaacga

SEQ ID NO: 202 - protein, 113 aa, Artificial Sequence
  Synthetic
DIQMTQSPLSLPVTPGEPASISCRSSQSLLHSHGYNYLDWYLQKPGQSPQLLIYLGSNRASGVPDRFSGGGSGTDFTLKISRVEAEDVGIYYCMQALQTPLTFGGGTKVEIKR

SEQ ID NO: 203 - DNA, 33 bp, Artificial Sequence
  Synthetic
cagagcctcctccatagtcatggatacaactat

SEQ ID NO: 204 - protein, 11 aa, Artificial Sequence
  Synthetic
QSLLHSHGYNY

SEQ ID NO: 205 - DNA, 9 bp, Artificial Sequence
  Synthetic
ttgggttct

SEQ ID NO: 206 - protein, 3 aa, Artificial Sequence
  Synthetic
LGS

SEQ ID NO: 207 - DNA, 27 bp, Artificial Sequence
  Synthetic
atgcaagctctacagactcctctcact

SEQ ID NO: 208 - protein, 9 aa, Artificial Sequence
  Synthetic
MQALQTPLT

SEQ ID NO: 209 - DNA, 375 bp, Artificial Sequence
  Synthetic
cagatcaccttgaaggagtctggtcctactctggtgaaaccctcacagaccctcacgctgacctgcaccttctctgggttctcactcagcactagtggagtgggtgtgggctggatccgtcagcccccaggaaaggccctggagtggcttgcactcatttattggaattctgataagcgctacagcccatctctgaagagcaggctcaccatcaccaaggacacctccaaaaaccaggtagtccttacaatgaccaacatggaccctgtggacacagccacatattactgtgcacacagacatgacagctcgtcctactacttctactacggtatggacgtctggggccaagggaccacggtcaccgtctcctca

SEQ ID NO: 210 - protein, 125 aa, Artificial Sequence
  Synthetic
QITLKESGPTLVKPSQTLTLTCTFSGFSLSTSGVGVGWIRQPPGKALEWLALIYWNSDKRYSPSLKSRLTITKDTSKNQVVLTMTNMDPVDTATYYCAHRHDSSSYYFYYGMDVWGQGTTVTVSS

SEQ ID NO: 211 - DNA, 336 bp, Artificial Sequence
  Synthetic
gatattgtgatgactcagtctccgctctccctgcccgtcacccctggagagccggcctccatctcctgcaggtctagtcagagcctcctccatagtcatggatacaactatttggattggtacctgcagaagccagggcagtctccacaactcctgatctatttgggttctaatcgggcctccggggtccctgacaggttcagtggcggtggatcaggcacagattttacactgaaaatcagcagagtggaggctgaggatgttgggatttattactgcatgcaagctctacagactcctctcactttcggcggagggaccaaggtggagatcaaa

SEQ ID NO: 212 - protein, 112 aa, Artificial Sequence
  Synthetic
DIVMTQSPLSLPVTPGEPASISCRSSQSLLHSHGYNYLDWYLQKPGQSPQLLIYLGSNRASGVPDRFSGGGSGTDFTLKISRVEAEDVGIYYCMQALQTPLTFGGGTKVEIK

SEQ ID NO: 213 - DNA, 375 bp, Artificial Sequence
  Synthetic
cagatcaccttgaaggagtctggtcctacgctggtgaaacccacacagaccctcacgctgacctgcaccttctctgggttctcactcagcactagtggagtgggtgtgggctggatccgtcagcccccaggaaaggccctggagtggcttgcactcatttattggaattctgataagcgctacagcccatctctgaagagcaggctcaccatcaccaaggacacctccaaaaaccaggtggtccttacaatgaccaacatggaccctgtggacacagccacatattactgtgcacacagacatgacagctcgtcctactacttctactacggtatggacgtctggggccaagggaccacggtcaccgtctcctca

SEQ ID NO: 214 - protein, 125 aa, Artificial Sequence
  Synthetic
QITLKESGPTLVKPTQTLTLTCTFSGFSLSTSGVGVGWIRQPPGKALEWLALIYWNSDKRYSPSLKSRLTITKDTSKNQVVLTMTNMDPVDTATYYCAHRHDSSSYYFYYGMDVWGQGTTVTVSS

SEQ ID NO: 215 - DNA, 336 bp, Artificial Sequence
  Synthetic
gatattgtgatgactcagtctccactctccctgcccgtcacccctggagagccggcctccatctcctgcaggtctagtcagagcctcctccatagtcatggatacaactatttggattggtacctgcagaagccagggcagtctccacagctcctgatctatttgggttctaatcgggcctccggggtccctgacaggttcagtggcagtggatcaggcacagattttacactgaaaatcagcagagtggaggctgaggatgttggggtttattactgcatgcaagctctacagactcctctcactttcggcggagggaccaaggtggagatcaaa

SEQ ID NO: 216 - protein, 112 aa, Artificial Sequence
  Synthetic
DIVMTQSPLSLPVTPGEPASISCRSSQSLLHSHGYNYLDWYLQKPGQSPQLLIYLGSNRASGVPDRFSGSGSGTDFTLKISRVEAEDVGVYYCMQALQTPLTFGGGTKVEIK

SEQ ID NO: 217 - DNA, 381 bp, Artificial Sequence
  Synthetic
gagatgcaactggtggagtctgggggaggcttggtccagcctggggggtccctgagactctcctgtgcagcctctggattcacctttagtagtcactggatgaagtgggtccgccaggctccagggaaggggctggagtgggtggccaacataaaccaagatggaagtgagaaatactatgtggactctgtgaagggccgattcaccatctccagagacaacgccaagaactcactgtttctgcaaatgaacagcctgagagccgaggacacggctgtgtattactgtgcgagagatattgtactaatggtctatgatatggactactactactacggtatggacgtctggggccaagggaccacggtcaccgtctcctca

SEQ ID NO: 218 - protein, 127 aa, Artificial Sequence
  Synthetic
EMQLVESGGGLVQPGGSLRLSCAASGFTFSSHWMKWVRQAPGKGLEWVANINQDGSEKYYVDSVKGRFTISRDNAKNSLFLQMNSLRAEDTAVYYCARDIVLMVYDMDYYYYGMDVWGQGTTVTVSS

SEQ ID NO: 219 - DNA, 24 bp, Artificial Sequence
  Synthetic
ggattcacctttagtagtcactgg

SEQ ID NO: 220 - protein, 8 aa, Artificial Sequence
  Synthetic
GFTFSSHW

SEQ ID NO: 221 - DNA, 24 bp, Artificial Sequence
  Synthetic
ataaaccaagatggaagtgagaaa

SEQ ID NO: 222 - protein, 8 aa, Artificial Sequence
  Synthetic
INQDGSEK

SEQ ID NO: 223 - DNA, 60 bp, Artificial Sequence
  Synthetic
gcgagagatattgtactaatggtctatgatatggactactactactacggtatggacgtc

SEQ ID NO: 224 - protein, 20 aa, Artificial Sequence
  Synthetic
ARDIVLMVYDMDYYYYGMDV

SEQ ID NO: 225 - DNA, 336 bp, Artificial Sequence
  Synthetic
gatattgtgatgactcagtctccactctccctgcccgtcacccctggagagccggcctccatctcctgcaggtctagtcagagcctcctgcatagtaatggaaacaactatttggattggtacctgcagaagccagggcagtctccacagctcctgatctatttgggttctaatcgggcctccggggtccctgacaggttcagtggcagtggatcaggcacagattttacactgaaaatcagcagagtggaggctgaggatgttggggtttattactgcatgcaaactctacaaactccgctcactttcggcggagggaccaaggtggagatcaaa

SEQ ID NO: 226 - protein, 112 aa, Artificial Sequence
  Synthetic
DIVMTQSPLSLPVTPGEPASISCRSSQSLLHSNGNNYLDWYLQKPGQSPQLLIYLGSNRASGVPDRFSGSGSGTDFTLKISRVEAEDVGVYYCMQTLQTPLTFGGGTKVEIK

SEQ ID NO: 227 - DNA, 33 bp, Artificial Sequence
  Synthetic
cagagcctcctgcatagtaatggaaacaactat

SEQ ID NO: 228 - protein, 11 aa, Artificial Sequence
  Synthetic
QSLLHSNGNNY

SEQ ID NO: 229 - DNA, 9 bp, Artificial Sequence
  Synthetic
ttgggttct

SEQ ID NO: 230 - protein, 3 aa, Artificial Sequence
  Synthetic
LGS

SEQ ID NO: 231 - DNA, 27 bp, Artificial Sequence
  Synthetic
atgcaaactctacaaactccgctcact

SEQ ID NO: 232 - protein, 9 aa, Artificial Sequence
  Synthetic
MQTLQTPLT

SEQ ID NO: 233 - DNA, 381 bp, Artificial Sequence
  Synthetic
gaggtgcagctggtggagtctgggggaggcttggtccagcctggggggtccctgagactctcctgtgcagcctctggattcacctttagtagtcactggatgaagtgggtccgccaggctccagggaaggggctggagtgggtggccaacataaaccaagatggaagtgagaaatactatgtggactctgtgaagggccgattcaccatctccagagacaacgccaagaactcactgtttctgcaaatgaacagcctgagagccgaggacacggctgtgtattactgtgcgagagatattgtactaatggtctatgatatggactactactactacggtatggacgtctggggccaagggaccacggtcaccgtctcctca

SEQ ID NO: 234 - protein, 127 aa, Artificial Sequence
  Synthetic
EVQLVESGGGLVQPGGSLRLSCAASGFTFSSHWMKWVRQAPGKGLEWVANINQDGSEKYYVDSVKGRFTISRDNAKNSLFLQMNSLRAEDTAVYYCARDIVLMVYDMDYYYYGMDVWGQGTTVTVSS

SEQ ID NO: 235 - DNA, 336 bp, Artificial Sequence; identical to SEQ ID NO: 225
  Synthetic

SEQ ID NO: 236 - protein, 112 aa, Artificial Sequence; identical to SEQ ID NO: 226
  Synthetic

SEQ ID NO: 237 - DNA, 381 bp, Artificial Sequence
  Synthetic
gaggtgcagctggtggagtctgggggaggcttggtccagcctggggggtccctgagactctcctgtgcagcctctggattcacctttagtagtcactggatgagctgggtccgccaggctccagggaaggggctggagtgggtggccaacataaaccaagatggaagtgagaaatactatgtggactctgtgaagggccgattcaccatctccagagacaacgccaagaactcactgtatctgcaaatgaacagcctgagagccgaggacacggctgtgtattactgtgcgagagatattgtactaatggtctatgatatggactactactactacggtatggacgtctgggggcaagggaccacggtcaccgtctcctca

SEQ ID NO: 238 - protein, 127 aa, Artificial Sequence
  Synthetic
EVQLVESGGGLVQPGGSLRLSCAASGFTFSSHWMSWVRQAPGKGLEWVANINQDGSEKYYVDSVKGRFTISRDNAKNSLYLQMNSLRAEDTAVYYCARDIVLMVYDMDYYYYGMDVWGQGTTVTVSS

SEQ ID NO: 239 - DNA, 336 bp, Artificial Sequence; identical to SEQ ID NO: 225
  Synthetic

SEQ ID NO: 240 - protein, 112 aa, Artificial Sequence; identical to SEQ ID NO: 226
  Synthetic

SEQ ID NO: 241 - DNA, 381 bp, Artificial Sequence
  Synthetic
caggtgcagctggtggagtctgggggaggcgtggtccagcctgggaggtccctgagactctcctgtgcagtctctggattcaccttcagtagctatggcatgcactgggtccgccaggctccaggcaaggggctggagtgggtggcagctatatcatatgatggaagtaataaatactatgtagactccgtgaagggccgattcaccatctccagagacaattccaagaaaacgctgtatctgcaaatgaacagcctgagagctgaggacacggctgtgtataattgtgcgaaaaatattgtactagtgatgtatgatatagactatcactactatgggatggacgtctggggccaagggaccacggtcaccgtctcctca

SEQ ID NO: 242 - protein, 127 aa, Artificial Sequence
  Synthetic
QVQLVESGGGVVQPGRSLRLSCAVSGFTFSSYGMHWVRQAPGKGLEWVAAISYDGSNKYYVDSVKGRFTISRDNSKKTLYLQMNSLRAEDTAVYNCAKNIVLVMYDIDYHYYGMDVWGQGTTVTVSS

SEQ ID NO: 243 - DNA, 24 bp, Artificial Sequence
  Synthetic
ggattcaccttcagtagctatggc

SEQ ID NO: 244 - protein, 8 aa, Artificial Sequence
  Synthetic
GFTFSSYG

SEQ ID NO: 245 - DNA, 24 bp, Artificial Sequence
  Synthetic
atatcatatgatggaagtaataaa

SEQ ID NO: 246 - protein, 8 aa, Artificial Sequence
  Synthetic
ISYDGSNK

SEQ ID NO: 247 - DNA, 60 bp, Artificial Sequence
  Synthetic
gcgaaaaatattgtactagtgatgtatgatatagactatcactactatgggatggacgtc

SEQ ID NO: 248 - protein, 20 aa, Artificial Sequence
  Synthetic
AKNIVLVMYDIDYHYYGMDV

SEQ ID NO: 249 - DNA, 336 bp, Artificial Sequence
  Synthetic
gatattgtgatgactcagtctccactctccctgcccgtcacccctggagagccggcctccatctcctgcaggtctagtcagagcctcctgcatagtaatggatacaactatttggattggtacctgcagaagccagggcagtctccacaactcctgatctatttgggttttaatcgggcctccggggtccctgacaggttcagtggcagtggatcaggcacagattttacactgaaaatcagcagagtggaggctgaggatgttggggtttattactgcatgcaagctctacaaactcctctcactttcggcggagggaccaaggtggagatcaga

SEQ ID NO: 250 - protein, 112 aa, Artificial Sequence
  Synthetic
DIVMTQSPLSLPVTPGEPASISCRSSQSLLHSNGYNYLDWYLQKPGQSPQLLIYLGFNRASGVPDRFSGSGSGTDFTLKISRVEAEDVGVYYCMQALQTPLTFGGGTKVEIR

SEQ ID NO: 251 - DNA, 33 bp, Artificial Sequence
  Synthetic
cagagcctcctgcatagtaatggatacaactat

SEQ ID NO: 252 - protein, 11 aa, Artificial Sequence
  Synthetic
QSLLHSNGYNY

SEQ ID NO: 253 - DNA, 9 bp, Artificial Sequence
  Synthetic
ttgggtttt

SEQ ID NO: 254 - protein, 3 aa, Artificial Sequence
  Synthetic
LGF

SEQ ID NO: 255 - DNA, 27 bp, Artificial Sequence
  Synthetic
atgcaagctctacaaactcctctcact

SEQ ID NO: 256 - protein, 9 aa, Artificial Sequence
  Synthetic
MQALQTPLT

SEQ ID NO: 257 - DNA, 381 bp, Artificial Sequence; identical to SEQ ID NO: 241
  Synthetic

SEQ ID NO: 258 - protein, 127 aa, Artificial Sequence; identical to SEQ ID NO: 242
  Synthetic

SEQ ID NO: 259 - DNA, 336 bp, Artificial Sequence
  Synthetic
gatattgtgatgactcagtctccactctccctgcccgtcacccctggagagccggcctccatctcctgcaggtctagtcagagcctcctgcatagtaatggatacaactatttggattggtacctgcagaagccagggcagtctccacaactcctgatctatttgggttttaatcgggcctccggggtccctgacaggttcagtggcagtggatcaggcacagattttacactgaaaatcagcagagtggaggctgaggatgttggggtttattactgcatgcaagctctacaaactcctctcactttcggcggagggaccaaggtggagatcaaa

SEQ ID NO: 260 - protein, 112 aa, Artificial Sequence
  Synthetic
DIVMTQSPLSLPVTPGEPASISCRSSQSLLHSNGYNYLDWYLQKPGQSPQLLIYLGFNRASGVPDRFSGSGSGTDFTLKISRVEAEDVGVYYCMQALQTPLTFGGGTKVEIK

SEQ ID NO: 261 - DNA, 381 bp, Artificial Sequence
  Synthetic
caggtgcagctggtggagtctgggggaggcgtggtccagcctgggaggtccctgagactctcctgtgcagcctctggattcaccttcagtagctatggcatgcactgggtccgccaggctccaggcaaggggctggagtgggtggcagttatatcatatgatggaagtaataaatactatgcagactccgtgaagggccgattcaccatctccagagacaattccaagaacacgctgtatctgcaaatgaacagcctgagagctgaggacacggctgtgtattactgtgcgaaaaatattgtactagtgatgtatgatatagactatcactactatgggatggacgtctgggggcaagggaccacggtcaccgtctcctca

SEQ ID NO: 262 - protein, 127 aa, Artificial Sequence
  Synthetic
QVQLVESGGGVVQPGRSLRLSCAASGFTFSSYGMHWVRQAPGKGLEWVAVISYDGSNKYYADSVKGRFTISRDNSKNTLYLQMNSLRAEDTAVYYCAKNIVLVMYDIDYHYYGMDVWGQGTTVTVSS

SEQ ID NO: 263 - DNA, 336 bp, Artificial Sequence
  Synthetic
gatattgtgatgactcagtctccactctccctgcccgtcacccctggagagccggcctccatctcctgcaggtctagtcagagcctcctgcatagtaatggatacaactatttggattggtacctgcagaagccagggcagtctccacagctcctgatctatttgggttttaatcgggcctccggggtccctgacaggttcagtggcagtggatcaggcacagattttacactgaaaatcagcagagtggaggctgaggatgttggggtttattactgcatgcaagctctacaaactcctctcactttcggcggagggaccaaggtggagatcaaa

SEQ ID NO: 264 - protein, 112 aa, Artificial Sequence; identical to SEQ ID NO: 260
  Synthetic

SEQ ID NO: 265 - DNA, 381 bp, Artificial Sequence; identical to SEQ ID NO: 241
  Synthetic

SEQ ID NO: 266 - protein, 127 aa, Artificial Sequence; identical to SEQ ID NO: 242
  Synthetic

SEQ ID NO: 267 - DNA, 24 bp, Artificial Sequence
  Synthetic
ggattcaccttcagtagctatggc

SEQ ID NO: 268 - protein, 8 aa, Artificial Sequence
  Synthetic
GFTFSSYG

SEQ ID NO: 269 - DNA, 24 bp, Artificial Sequence
  Synthetic
atatcatatgatggaagtaataaa

SEQ ID NO: 270 - protein, 8 aa, Artificial Sequence
  Synthetic
ISYDGSNK

SEQ ID NO: 271 - DNA, 60 bp, Artificial Sequence; identical to SEQ ID NO: 247
  Synthetic

SEQ ID NO: 272 - protein, 20 aa, Artificial Sequence
  Synthetic
AKNIVLVMYDIDYHYYGMDV

SEQ ID NO: 273 - DNA, 336 bp, Artificial Sequence; identical to SEQ ID NO: 249
  Synthetic

SEQ ID NO: 274 - protein, 112 aa, Artificial Sequence; identical to SEQ ID NO: 250
  Synthetic

SEQ ID NO: 275 - DNA, 33 bp, Artificial Sequence; identical to SEQ ID NO: 251
  Synthetic

SEQ ID NO: 276 - protein, 11 aa, Artificial Sequence
  Synthetic
QSLLHSNGYNY

SEQ ID NO: 277 - DNA, 9 bp, Artificial Sequence
  Synthetic
ttgggtttt

SEQ ID NO: 278 - protein, 3 aa, Artificial Sequence
  Synthetic
LGF

SEQ ID NO: 279 - DNA, 27 bp, Artificial Sequence
  Synthetic
atgcaagctctacaaactcctctcact

SEQ ID NO: 280 - protein, 9 aa, Artificial Sequence
  Synthetic
MQALQTPLT

SEQ ID NO: 281 - DNA, 381 bp, Artificial Sequence; identical to SEQ ID NO: 241
  Synthetic

SEQ ID NO: 282 - protein, 127 aa, Artificial Sequence; identical to SEQ ID NO: 242
  Synthetic

SEQ ID NO: 283 - DNA, 336 bp, Artificial Sequence; identical to SEQ ID NO: 259
  Synthetic

SEQ ID NO: 284 - protein, 112 aa, Artificial Sequence; identical to SEQ ID NO: 260
  Synthetic

SEQ ID NO: 285 - DNA, 381 bp, Artificial Sequence; identical to SEQ ID NO: 261
  Synthetic

SEQ ID NO: 286 - protein, 127 aa, Artificial Sequence; identical to SEQ ID NO: 262
  Synthetic

SEQ ID NO: 287 - DNA, 336 bp, Artificial Sequence; identical to SEQ ID NO: 263
  Synthetic

SEQ ID NO: 288 - protein, 112 aa, Artificial Sequence; identical to SEQ ID NO: 260
  Synthetic

SEQ ID NO: 289 - DNA, 372 bp, Artificial Sequence
  Synthetic
cagatcaccttgaaggagtctggtcctacgctggtaaaacccacacagaccctcacgctgacctgcaccttctctgggttctcactcagcgctagtggagtgggtgtgggctggttccgtcagcccccaggaaaggccctggagtggcttgcactcatttattggaatgatgataagcgttacagcccatctctaaagaacagcctcaccatcaccaaggacacctccaaaaaccaggtggtccttacaatgaccaacatggaccctgtggacacagccacatattactgtgcacacagaatacatctatggtcctacttctactacggtatggacgtctggggccaagggaccacggtcaccgtctcctca

SEQ ID NO: 290 - protein, 124 aa, Artificial Sequence
  Synthetic
QITLKESGPTLVKPTQTLTLTCTFSGFSLSASGVGVGWFRQPPGKALEWLALIYWNDDKRYSPSLKNSLTITKDTSKNQVVLTMTNMDPVDTATYYCAHRIHLWSYFYYGMDVWGQGTTVTVSS

SEQ ID NO: 291 - DNA, 30 bp, Artificial Sequence
  Synthetic
gggttctcactcagcgctagtggagtgggt

SEQ ID NO: 292 - protein, 10 aa, Artificial Sequence
  Synthetic
GFSLSASGVG

SEQ ID NO: 293 - DNA, 21 bp, Artificial Sequence
  Synthetic
atttattggaatgatgataag

SEQ ID NO: 294 - protein, 7 aa, Artificial Sequence
  Synthetic
IYWNDDK

SEQ ID NO: 295 - DNA, 48 bp, Artificial Sequence
  Synthetic
gcacacagaatacatctatggtcctacttctactacggtatggacgtc

SEQ ID NO: 296 - protein, 16 aa, Artificial Sequence
  Synthetic
AHRIHLWSYFYYGMDV

SEQ ID NO: 297 - DNA, 336 bp, Artificial Sequence
  Synthetic
gatattgtgatgactcagtctccactctccctgcccgtcacccctggagagccggcctccatctcctgcaggtctagtcagactctcctgcatagtaatggatacaactatttcgattggtacctgcagaagccagggcagtctccacagctcctgatctatttgggttctaatcgggcctccggggtccctgacagattcagtggcagtggatcaggcacagattttacactgaaaatcagcagagtggaggctgaggatgttggaatttattactgcatgcaagctctacaaactcctctcactttcggcggagggaccaaggtggagatcaga

SEQ ID NO: 298 - protein, 112 aa, Artificial Sequence
  Synthetic
DIVMTQSPLSLPVTPGEPASISCRSSQTLLHSNGYNYFDWYLQKPGQSPQLLIYLGSNRASGVPDRFSGSGSGTDFTLKISRVEAEDVGIYYCMQALQTPLTFGGGTKVEIR

SEQ ID NO: 299 - DNA, 33 bp, Artificial Sequence
  Synthetic
cagactctcctgcatagtaatggatacaactat

SEQ ID NO: 300 - protein, 11 aa, Artificial Sequence
  Synthetic
QTLLHSNGYNY

SEQ ID NO: 301 - DNA, 9 bp, Artificial Sequence
  Synthetic
ttgggttct

SEQ ID NO: 302 - protein, 3 aa, Artificial Sequence
  Synthetic
LGS

SEQ ID NO: 303 - DNA, 27 bp, Artificial Sequence
  Synthetic
atgcaagctctacaaactcctctcact

SEQ ID NO: 304 - protein, 9 aa, Artificial Sequence
  Synthetic
MQALQTPLT

SEQ ID NO: 305 - DNA, 372 bp, Artificial Sequence; identical to SEQ ID NO: 289
  Synthetic

SEQ ID NO: 306 - protein, 124 aa, Artificial Sequence; identical to SEQ ID NO: 290
  Synthetic

SEQ ID NO: 307 - DNA, 336 bp, Artificial Sequence
  Synthetic
gatattgtgatgactcagtctccactctccctgcccgtcacccctggagagccggcctccatctcctgcaggtctagtcagactctcctgcatagtaatggatacaactatttcgattggtacctgcagaagccagggcagtctccacagctcctgatctatttgggttctaatcgggcctccggggtccctgacagattcagtggcagtggatcaggcacagattttacactgaaaatcagcagagtggaggctgaggatgttggaatttattactgcatgcaagctctacaaactcctctcactttcggcggagggaccaaggtggagatcaaa

SEQ ID NO: 308 - protein, 112 aa, Artificial Sequence
  Synthetic
DIVMTQSPLSLPVTPGEPASISCRSSQTLLHSNGYNYFDWYLQKPGQSPQLLIYLGSNRASGVPDRFSGSGSGTDFTLKISRVEAEDVGIYYCMQALQTPLTFGGGTKVEIK

SEQ ID NO: 309 - DNA, 372 bp, Artificial Sequence
  Synthetic
cagatcaccttgaaggagtctggtcctacgctggtgaaacccacacagaccctcacgctgacctgcaccttctctgggttctcactcagcgctagtggagtgggtgtgggctggatccgtcagcccccaggaaaggccctggagtggcttgcactcatttattggaatgatgataagcgctacagcccatctctgaagagcaggctcaccatcaccaaggacacctccaaaaaccaggtggtccttacaatgaccaacatggaccctgtggacacagccacatattactgtgcacacagaatacatctatggtcctacttctactacggtatggacgtctgggggcaagggaccacggtcaccgtctcctca

SEQ ID NO: 310 - protein, 124 aa, Artificial Sequence
  Synthetic
QITLKESGPTLVKPTQTLTLTCTFSGFSLSASGVGVGWIRQPPGKALEWLALIYWNDDKRYSPSLKSRLTITKDTSKNQVVLTMTNMDPVDTATYYCAHRIHLWSYFYYGMDVWGQGTTVTVSS

SEQ ID NO: 311 - DNA, 336 bp, Artificial Sequence
  Synthetic
gatattgtgatgactcagtctccactctccctgcccgtcacccctggagagccggcctccatctcctgcaggtctagtcagactctcctgcatagtaatggatacaactatttggattggtacctgcagaagccagggcagtctccacagctcctgatctatttgggttctaatcgggcctccggggtccctgacaggttcagtggcagtggatcaggcacagattttacactgaaaatcagcagagtggaggctgaggatgttggggtttattactgcatgcaagctctacaaactcctctcactttcggcggagggaccaaggtggagatcaaa

SEQ ID NO: 312 - protein, 112 aa, Artificial Sequence
  Synthetic
DIVMTQSPLSLPVTPGEPASISCRSSQTLLHSNGYNYLDWYLQKPGQSPQLLIYLGSNRASGVPDRFSGSGSGTDFTLKISRVEAEDVGVYYCMQALQTPLTFGGGTKVEIK

SEQ ID NO: 313 - DNA, 381 bp, Artificial Sequence
  Synthetic
caggttcagctggtgcagtctggacctgaggtgaagaaccctggggcctcagtgaaggtctcctgcaaggcttctggttacacctttaccacctatggtatcagttgggtacgacaggcccctggacaagggcttgagtggatgggatggatcagcggttacaatggtaaaacaaacgatgcacagaagttccaggacagagtcgccatgaccacagacacatccacgagcacagcctacatggagctgaggagcctgagatctgacgacacggccatttattactgttcgagagatcgtttagtagtaccacctgcccttaattattcctactacgttatggacgtctggggccaagggaccacggtcaccgtctcctca

SEQ ID NO: 314 - protein, 127 aa, Artificial Sequence
  Synthetic
QVQLVQSGPEVKNPGASVKVSCKASGYTFTTYGISWVRQAPGQGLEWMGWISGYNGKTNDAQKFQDRVAMTTDTSTSTAYMELRSLRSDDTAIYYCSRDRLVVPPALNYSYYVMDVWGQGTTVTVSS

SEQ ID NO: 315 - DNA, 24 bp, Artificial Sequence
  Synthetic
ggttacacctttaccacctatggt

SEQ ID NO: 316 - protein, 8 aa, Artificial Sequence
  Synthetic
GYTFTTYG

SEQ ID NO: 317 - DNA, 24 bp, Artificial Sequence
  Synthetic
atcagcggttacaatggtaaaaca

SEQ ID NO: 318 - protein, 8 aa, Artificial Sequence
  Synthetic
ISGYNGKT

SEQ ID NO: 319 - DNA, 60 bp, Artificial Sequence
  Synthetic
tcgagagatcgtttagtagtaccacctgcccttaattattcctactacgttatggacgtc

SEQ ID NO: 320 - protein, 20 aa, Artificial Sequence
  Synthetic
SRDRLVVPPALNYSYYVMDV

SEQ ID NO: 321 - DNA, 336 bp, Artificial Sequence
  Synthetic
gatgttgtgatgactcagtctccactctccctgcccgtcacccttggacagccggcctccatctcctgcaggtctagtcaaagcctcgtatacagtgatggaaacacctacttgaattggtctcagcagaggccaggtcaatctccaaggcgcctaatttataaggtttctaaccgggactctggggtcccagacagattcagcggcagtgggtcaggcactgatttcacactgaaaatcagcagggtggaggctgaggatgttggggtttattactgcatgcaaggtacacactggccgtacacttttggccaggggaccaagctggagatcaaa

SEQ ID NO: 322 - protein, 112 aa, Artificial Sequence
  Synthetic
DVVMTQSPLSLPVTLGQPASISCRSSQSLVYSDGNTYLNWSQQRPGQSPRRLIYKVSNRDSGVPDRFSGSGSGTDFTLKISRVEAEDVGVYYCMQGTHWPYTFGQGTKLEIK

SEQ ID NO: 323 - DNA, 33 bp, Artificial Sequence
  Synthetic
caaagcctcgtatacagtgatggaaacacctac

SEQ ID NO: 324 - protein, 11 aa, Artificial Sequence
  Synthetic
QSLVYSDGNTY

SEQ ID NO: 325 - DNA, 9 bp, Artificial Sequence
  Synthetic
aaggtttct

SEQ ID NO: 326 - protein, 3 aa, Artificial Sequence
  Synthetic
KVS

SEQ ID NO: 327 - DNA, 27 bp, Artificial Sequence
  Synthetic
atgcaaggtacacactggccgtacact

SEQ ID NO: 328 - protein, 9 aa, Artificial Sequence
  Synthetic
MQGTHWPYT

SEQ ID NO: 329 - DNA, 381 bp, Artificial Sequence; identical to SEQ ID NO: 313
  Synthetic

SEQ ID NO: 330 - protein, 127 aa, Artificial Sequence; identical to SEQ ID NO: 314
  Synthetic

SEQ ID NO: 331 - DNA, 336 bp, Artificial Sequence; identical to SEQ ID NO: 321
  Synthetic

SEQ ID NO: 332 - protein, 112 aa, Artificial Sequence; identical to SEQ ID NO: 322
  Synthetic

SEQ ID NO: 333 - DNA, 381 bp, Artificial Sequence
  Synthetic
caggttcagctggtgcagtctggagctgaggtgaagaagcctggggcctcagtgaaggtctcctgcaaggcttctggttacacctttaccacctatggtatcagctgggtgcgacaggcccctggacaagggcttgagtggatgggatggatcagcggttacaatggtaaaacaaactatgcacagaagctccagggcagagtcaccatgaccacagacacatccacgagcacagcctacatggagctgaggagcctgagatctgacgacacggccgtgtattactgttcgagagatcgtttagtagtaccacctgcccttaattattcctactacgttatggacgtctgggggcaagggaccacggtcaccgtctcctca

SEQ ID NO: 334 - protein, 127 aa, Artificial Sequence
  Synthetic
QVQLVQSGAEVKKPGASVKVSCKASGYTFTTYGISWVRQAPGQGLEWMGWISGYNGKTNYAQKLQGRVTMTTDTSTSTAYMELRSLRSDDTAVYYCSRDRLVVPPALNYSYYVMDVWGQGTTVTVSS

SEQ ID NO: 335 - DNA, 336 bp, Artificial Sequence
  Synthetic
gatgttgtgatgactcagtctccactctccctgcccgtcacccttggacagccggcctccatctcctgcaggtctagtcaaagcctcgtatacagtgatggaaacacctacttgaattggtttcagcagaggccaggccaatctccaaggcgcctaatttataaggtttctaaccgggactctggggtcccagacagattcagcggcagtgggtcaggcactgatttcacactgaaaatcagcagggtggaggctgaggatgttggggtttattactgcatgcaaggtacacactggccgtacacttttggccaggggaccaagctggagatcaaa

SEQ ID NO: 336 - protein, 112 aa, Artificial Sequence
  Synthetic
DVVMTQSPLSLPVTLGQPASISCRSSQSLVYSDGNTYLNWFQQRPGQSPRRLIYKVSNRDSGVPDRFSGSGSGTDFTLKISRVEAEDVGVYYCMQGTHWPYTFGQGTKLEIK

SEQ ID NO: 337 - DNA, 354 bp, Artificial Sequence
  Synthetic
gaggtgcagctggtggagtctgggggaggcctggtcaagcctggggggtccctgagactctcctgtgcagcctctggattcaccttcagtagctatagcatggactgggtccgccaggctccagggaaggggctggagtgggtctcatccattagtagtagtagtagttacatatactacgcagactctgtgaagggccgattcaccatctccagagacaccgccaagaactcactgtatctgcaaatgaacagcctgagagacgaggacacggctgtttattactgtgcgagagagggcagtagcagactttttgactactggggccagggaaccctggtcaccgtctcctca

SEQ ID NO: 338 - protein, 118 aa, Artificial Sequence
  Synthetic
EVQLVESGGGLVKPGGSLRLSCAASGFTFSSYSMDWVRQAPGKGLEWVSSISSSSSYIYYADSVKGRFTISRDTAKNSLYLQMNSLRDEDTAVYYCAREGSSRLFDYWGQGTLVTVSS

SEQ ID NO: 339 - DNA, 24 bp, Artificial Sequence
  Synthetic
ggattcaccttcagtagctatagc

SEQ ID NO: 340 - protein, 8 aa, Artificial Sequence
  Synthetic
GFTFSSYS

SEQ ID NO: 341 - DNA, 24 bp, Artificial Sequence
  Synthetic
attagtagtagtagtagttacata

SEQ ID NO: 342 - protein, 8 aa, Artificial Sequence
  Synthetic
ISSSSSYI

SEQ ID NO: 343 - DNA, 33 bp, Artificial Sequence
  Synthetic
gcgagagagggcagtagcagactttttgactac

SEQ ID NO: 344 - protein, 11 aa, Artificial Sequence
  Synthetic
AREGSSRLFDY

SEQ ID NO: 345 - DNA, 321 bp, Artificial Sequence
  Synthetic
gacatccagatgacccagtctccttccaccctgtctgcatctgtaggagacagagtcaccatcacttgccgggccagtcagagtattagtagctggttggcctggtatcagcagagaccagggaaagcccctaagctcctgatctataaggcgtctagtttagaaggtggagtcccatcaaggttcagcggcagtggatctgggacagaattcactctcaccatcagcagcctgcagcctgaggattttgcaacttattactgccaacagtataatagttattggtacacttttggccaggggaccaagctggagatcaaa

SEQ ID NO: 346 - protein, 107 aa, Artificial Sequence
  Synthetic
DIQMTQSPSTLSASVGDRVTITCRASQSISSWLAWYQQRPGKAPKLLIYKASSLEGGVPSRFSGSGSGTEFTLTISSLQPEDFATYYCQQYNSYWYTFGQGTKLEIK

SEQ ID NO: 347 - DNA, 18 bp, Artificial Sequence
  Synthetic
cagagtattagtagctgg

SEQ ID NO: 348 - protein, 6 aa, Artificial Sequence
  Synthetic
QSISSW

SEQ ID NO: 349 - DNA, 9 bp, Artificial Sequence
  Synthetic
aaggcgtct

SEQ ID NO: 350 - protein, 3 aa, Artificial Sequence
  Synthetic
KAS

SEQ ID NO: 351 - DNA, 27 bp, Artificial Sequence
  Synthetic
caacagtataatagttattggtacact

SEQ ID NO: 352 - protein, 9 aa, Artificial Sequence
  Synthetic
QQYNSYWYT

SEQ ID NO: 353 - DNA, 354 bp, Artificial Sequence; identical to SEQ ID NO: 337
  Synthetic

SEQ ID NO: 354 - protein, 118 aa, Artificial Sequence; identical to SEQ ID NO: 338
  Synthetic

SEQ ID NO: 355 - DNA, 321 bp, Artificial Sequence; identical to SEQ ID NO: 345
  Synthetic

SEQ ID NO: 356 - protein, 107 aa, Artificial Sequence; identical to SEQ ID NO: 346
  Synthetic

SEQ ID NO: 357 - DNA, 354 bp, Artificial Sequence
  Synthetic
gaggtgcagctggtggagtctgggggaggcctggtcaagcctggggggtccctgagactctcctgtgcagcctctggattcaccttcagtagctatagcatgaactgggtccgccaggctccagggaaggggctggagtgggtctcatccattagtagtagtagtagttacatatactacgcagactcagtgaagggccgattcaccatctccagagacaacgccaagaactcactgtatctgcaaatgaacagcctgagagccgaggacacggctgtgtattactgtgcgagagagggcagtagcagactttttgactactggggccaaggaaccctggtcaccgtctcctca

SEQ ID NO: 358 - protein, 118 aa, Artificial Sequence
  Synthetic
EVQLVESGGGLVKPGGSLRLSCAASGFTFSSYSMNWVRQAPGKGLEWVSSISSSSSYIYYADSVKGRFTISRDNAKNSLYLQMNSLRAEDTAVYYCAREGSSRLFDYWGQGTLVTVSS

SEQ ID NO: 359 - DNA, 321 bp, Artificial Sequence
  Synthetic
gacatccagatgacccagtctccttccaccctgtctgcatctgtaggagacagagtcaccatcacttgccgggccagtcagagtattagtagctggttggcctggtatcagcagaaaccagggaaagcccctaagctcctgatctataaggcgtctagtttagaaagtggggtcccatcaaggttcagcggcagtggatctgggacagaattcactctcaccatcagcagcctgcagcctgatgattttgcaacttattactgccaacagtataatagttattggtacacttttggccaggggaccaagctggagatcaaa

SEQ ID NO: 360 - protein, 107 aa, Artificial Sequence
  Synthetic
DIQMTQSPSTLSASVGDRVTITCRASQSISSWLAWYQQKPGKAPKLLIYKASSLESGVPSRFSGSGSGTEFTLTISSLQPDDFATYYCQQYNSYWYTFGQGTKLEIK

SEQ ID NO: 361 - DNA, 384 bp, Artificial Sequence
  Synthetic
caggtgcacctggtggagtctgggggaggcttggtcaagcctggagggtccctgagactctcctgtgcagcctctggattcaccttcagtgaccactacatgagctggatccgccaggctccagggaaggggctggagtggatttcatacattagtaatgatggtggtaccaaatactatgtggactctgtggagggccgattcatcatttccagggacaacgccaagaactcattgtatctacatatgaacagcctcagagccgacgacacggccgtgtattactgtgcgagagatcagggatatattggctacgactcgtattattactattcctacggtatggacgtctggggccaagggaccacggtcaccgtcgcctca

SEQ ID NO: 362 - protein, 128 aa, Artificial Sequence
  Synthetic
QVHLVESGGGLVKPGGSLRLSCAASGFTFSDHYMSWIRQAPGKGLEWISYISNDGGTKYYVDSVEGRFIISRDNAKNSLYLHMNSLRADDTAVYYCARDQGYIGYDSYYYYSYGMDVWGQGTTVTVAS

SEQ ID NO: 363 - DNA, 24 bp, Artificial Sequence
  Synthetic
ggattcaccttcagtgaccactac

SEQ ID NO: 364 - protein, 8 aa, Artificial Sequence
  Synthetic
GFTFSDHY

SEQ ID NO: 365 - DNA, 24 bp, Artificial Sequence
  Synthetic
attagtaatgatggtggtaccaaa

SEQ ID NO: 366 - protein, 8 aa, Artificial Sequence
  Synthetic
ISNDGGTK

SEQ ID NO: 367 - DNA, 63 bp, Artificial Sequence
  Synthetic
gcgagagatcagggatatattggctacgactcgtattattactattcctacggtatggacgtc

SEQ ID NO: 368 - protein, 21 aa, Artificial Sequence
  Synthetic
ARDQGYIGYDSYYYYSYGMDV

SEQ ID NO: 369 - DNA, 321 bp, Artificial Sequence
  Synthetic
aaaattgtgttgacgcagtctccaggcaccctgcctttgtttccaggggaaagagccaccctctcctgtagggccagtcagagtgttaacaacaaattcttagcctggtaccagcagaaatctggccaggctcccaggctcctcatctatggtgcatccagcagggccactggcatcccagacaggttcagtggcagtgggtctgggaccgacttcactctcaccatcagcggactggagcctgaagattttgaagtgtattattgtcaagtatatggtaactcactcactctcggcggagggaccaaggtggagatcaag

SEQ ID NO: 370 - protein, 107 aa, Artificial Sequence
  Synthetic
KIVLTQSPGTLPLFPGERATLSCRASQSVNNKFLAWYQQKSGQAPRLLIYGASSRATGIPDRFSGSGSGTDFTLTISGLEPEDFEVYYCQVYGNSLTLGGGTKVEIK

SEQ ID NO: 371 - DNA, 21 bp, Artificial Sequence
  Synthetic
cagagtgttaacaacaaattc

SEQ ID NO: 372 - protein, 7 aa, Artificial Sequence
  Synthetic
QSVNNKF

SEQ ID NO: 373 - DNA, 9 bp, Artificial Sequence
  Synthetic
ggtgcatcc

SEQ ID NO: 374 - protein, 3 aa, Artificial Sequence
  Synthetic
GAS

SEQ ID NO: 375 - DNA, 24 bp, Artificial Sequence
  Synthetic
caagtatatggtaactcactcact

SEQ ID NO: 376 - protein, 8 aa, Artificial Sequence
  Synthetic
QVYGNSLT

SEQ ID NO: 377 - DNA, 384 bp, Artificial Sequence
  Synthetic
caggtgcagctggtggagtctgggggaggcttggtcaagcctggagggtccctgagactctcctgtgcagcctctggattcaccttcagtgaccactacatgagctggatccgccaggctccagggaaggggctggagtggatttcatacattagtaatgatggtggtaccaaatactatgtggactctgtggagggccgattcatcatttccagggacaacgccaagaactcattgtatctacatatgaacagcctcagagccgacgacacggccgtgtattactgtgcgagagatcagggatatattggctacgactcgtattattactattcctacggtatggacgtctggggccaagggaccacggtcaccgtctcctca

SEQ ID NO: 378 - protein, 128 aa, Artificial Sequence
  Synthetic
QVQLVESGGGLVKPGGSLRLSCAASGFTFSDHYMSWIRQAPGKGLEWISYISNDGGTKYYVDSVEGRFIISRDNAKNSLYLHMNSLRADDTAVYYCARDQGYIGYDSYYYYSYGMDVWGQGTTVTVSS

SEQ ID NO: 379 - DNA, 321 bp, Artificial Sequence
  Synthetic
gaaattgtgttgacgcagtctccaggcaccctgcctttgtttccaggggaaagagccaccctctcctgtagggccagtcagagtgttaacaacaaattcttagcctggtaccagcagaaatctggccaggctcccaggctcctcatctatggtgcatccagcagggccactggcatcccagacaggttcagtggcagtgggtctgggaccgacttcactctcaccatcagcggactggagcctgaagattttgaagtgtattattgtcaagtatatggtaactcactcactctcggcggagggaccaaggtggagatcaaa

SEQ ID NO: 380 - protein, 107 aa, Artificial Sequence
  Synthetic
EIVLTQSPGTLPLFPGERATLSCRASQSVNNKFLAWYQQKSGQAPRLLIYGASSRATGIPDRFSGSGSGTDFTLTISGLEPEDFEVYYCQVYGNSLTLGGGTKVEIK

SEQ ID NO: 381 - DNA, 384 bp, Artificial Sequence
  Synthetic
caggtgcagctggtggagtctgggggaggcttggtcaagcctggagggtccctgagactctcctgtgcagcctctggattcaccttcagtgaccactacatgagctggatccgccaggctccagggaaggggctggagtgggtttcatacattagtaatgatggtggtaccaaatactacgcagactctgtgaagggccgattcaccatctccagggacaacgccaagaactcactgtatctgcaaatgaacagcctgagagccgaggacacggccgtgtattactgtgcgagagatcagggatatattggctacgactcgtattattactattcctacggtatggacgtctgggggcaagggaccacggtcaccgtctcctca

SEQ ID NO: 382 - protein, 128 aa, Artificial Sequence
  Synthetic
QVQLVESGGGLVKPGGSLRLSCAASGFTFSDHYMSWIRQAPGKGLEWVSYISNDGGTKYYADSVKGRFTISRDNAKNSLYLQMNSLRAEDTAVYYCARDQGYIGYDSYYYYSYGMDVWGQGTTVTVSS

SEQ ID NO: 383 - DNA, 321 bp, Artificial Sequence
  Synthetic
gaaattgtgttgacgcagtctccaggcaccctgtctttgtctccaggggaaagagccaccctctcctgcagggccagtcagagtgttaacaacaaattcttagcctggtaccagcagaaacctggccaggctcccaggctcctcatctatggtgcatccagcagggccactggcatcccagacaggttcagtggcagtgggtctgggacagacttcactctcaccatcagcagactggagcctgaagattttgcagtgtattactgtcaagtatatggtaactcactcactttcggcggagggaccaaggtggagatcaaa

SEQ ID NO: 384 - protein, 107 aa, Artificial Sequence
  Synthetic
EIVLTQSPGTLSLSPGERATLSCRASQSVNNKFLAWYQQKPGQAPRLLIYGASSRATGIPDRFSGSGSGTDFTLTISRLEPEDFAVYYCQVYGNSLTFGGGTKVEIK

SEQ ID NO: 385 - DNA, 360 bp, Artificial Sequence
  Synthetic
gaggtgcagaaggtggagtctgggggaggcctggtcaagccgggggggtccctgagactctcctgtacagcctctggattcaccttcagtacttataacatgaattgggtccgccaggctccagggaagggactggagtgggtctcatccattaggagtagtagtaattacatatactacgcagactcagtgaagggccgattcaccatctccagagacaacgccaagaattcactgtatctgcaaatgaacagcctgagagccgatgacacggctgtgtattactgtgcgagagatggcagcagttggtacgactactctgactactggggccagggaaccctggtcaccgtctcctca

SEQ ID NO: 386 - protein, 120 aa, Artificial Sequence
  Synthetic
EVQKVESGGGLVKPGGSLRLSCTASGFTFSTYNMNWVRQAPGKGLEWVSSIRSSSNYIYYADSVKGRFTISRDNAKNSLYLQMNSLRADDTAVYYCARDGSSWYDYSDYWGQGTLVTVSS

SEQ ID NO: 387 - DNA, 24 bp, Artificial Sequence
  Synthetic
ggattcaccttcagtacttataac

SEQ ID NO: 388 - protein, 8 aa, Artificial Sequence
  Synthetic
GFTFSTYN

SEQ ID NO: 389 - DNA, 24 bp, Artificial Sequence
  Synthetic
attaggagtagtagtaattacata

SEQ ID NO: 390 - protein, 8 aa, Artificial Sequence
  Synthetic
IRSSSNYI

SEQ ID NO: 391 - DNA, 39 bp, Artificial Sequence
  Synthetic
gcgagagatggcagcagttggtacgactactctgactac

SEQ ID NO: 392 - protein, 13 aa, Artificial Sequence
  Synthetic
ARDGSSWYDYSDY

SEQ ID NO: 393 - DNA, 321 bp, Artificial Sequence
  Synthetic
gacatccagatgacccagtctccttccaccctgtctgcatctgtaggagacagagtcaccatcacttgccgggccagtcagagtattagtagctggttggcctggtatcaacagataccagggaaagcccctaaactcctgatctataaggcgtctagtttagaaaatggggtcccatcaaggttcagcggcagtggatctgggacagaattcactctcatcatcagcagcctgcagcctgatgattttgcaacttattactgccaacagtatattagttattctcggacgttcggccaagggaccaaggtggaaatcaaa

SEQ ID NO: 394 - protein, 107 aa, Artificial Sequence
  Synthetic
DIQMTQSPSTLSASVGDRVTITCRASQSISSWLAWYQQIPGKAPKLLIYKASSLENGVPSRFSGSGSGTEFTLIISSLQPDDFATYYCQQYISYSRTFGQGTKVEIK

SEQ ID NO: 395 - DNA, 18 bp, Artificial Sequence
  Synthetic
cagagtattagtagctgg

SEQ ID NO: 396 - protein, 6 aa, Artificial Sequence
  Synthetic
QSISSW

SEQ ID NO: 397 - DNA, 9 bp, Artificial Sequence
  Synthetic
aaggcgtct

SEQ ID NO: 398 - protein, 3 aa, Artificial Sequence
  Synthetic
KAS

SEQ ID NO: 399 - DNA, 27 bp, Artificial Sequence
  Synthetic
caacagtatattagttattctcggacg

SEQ ID NO: 400 - protein, 9 aa, Artificial Sequence
  Synthetic
QQYISYSRT

SEQ ID NO: 401 - DNA, 360 bp, Artificial Sequence
  Synthetic
gaggtgcagctggtggagtctgggggaggcctggtcaagccgggggggtccctgagactctcctgtacagcctctggattcaccttcagtacttataacatgaattgggtccgccaggctccagggaagggactggagtgggtctcatccattaggagtagtagtaattacatatactacgcagactcagtgaagggccgattcaccatctccagagacaacgccaagaattcactgtatctgcaaatgaacagcctgagagccgatgacacggctgtgtattactgtgcgagagatggcagcagttggtacgactactctgactactggggccagggaaccctggtcaccgtctcctca

SEQ ID NO: 402 - protein, 120 aa, Artificial Sequence
  Synthetic
EVQLVESGGGLVKPGGSLRLSCTASGFTFSTYNMNWVRQAPGKGLEWVSSIRSSSNYIYYADSVKGRFTISRDNAKNSLYLQMNSLRADDTAVYYCARDGSSWYDYSDYWGQGTLVTVSS

SEQ ID NO: 403 - DNA, 321 bp, Artificial Sequence; identical to SEQ ID NO: 393
  Synthetic

SEQ ID NO: 404 - protein, 107 aa, Artificial Sequence; identical to SEQ ID NO: 394
  Synthetic

SEQ ID NO: 405 - DNA, 360 bp, Artificial Sequence
  Synthetic
gaggtgcagctggtggagtctgggggaggcctggtcaagcctggggggtccctgagactctcctgtgcagcctctggattcaccttcagtacttataacatgaactgggtccgccaggctccagggaaggggctggagtgggtctcatccattaggagtagtagtaattacatatactacgcagactcagtgaagggccgattcaccatctccagagacaacgccaagaactcactgtatctgcaaatgaacagcctgagagccgaggacacggctgtgtattactgtgcgagagatggcagcagttggtacgactactctgactactggggccaaggaaccctggtcaccgtctcctca

SEQ ID NO: 406 - protein, 120 aa, Artificial Sequence
  Synthetic
EVQLVESGGGLVKPGGSLRLSCAASGFTFSTYNMNWVRQAPGKGLEWVSSIRSSSNYIYYADSVKGRFTISRDNAKNSLYLQMNSLRAEDTAVYYCARDGSSWYDYSDYWGQGTLVTVSS

SEQ ID NO: 407 - DNA, 321 bp, Artificial Sequence
  Synthetic
gacatccagatgacccagtctccttccaccctgtctgcatctgtaggagacagagtcaccatcacttgccgggccagtcagagtattagtagctggttggcctggtatcagcagaaaccagggaaagcccctaagctcctgatctataaggcgtctagtttagaaagtggggtcccatcaaggttcagcggcagtggatctgggacagaattcactctcaccatcagcagcctgcagcctgatgattttgcaacttattactgccaacagtatattagttattctcggacgttcggccaagggaccaaggtggaaatcaaa

SEQ ID NO: 408 - protein, 107 aa, Artificial Sequence
  Synthetic
DIQMTQSPSTLSASVGDRVTITCRASQSISSWLAWYQQKPGKAPKLLIYKASSLESGVPSRFSGSGSGTEFTLTISSLQPDDFATYYCQQYISYSRTFGQGTKVEIK

SEQ ID NO: 409 - DNA, 360 bp, Artificial Sequence; identical to SEQ ID NO: 401
  Synthetic

SEQ ID NO: 410 - protein, 120 aa, Artificial Sequence; identical to SEQ ID NO: 402
  Synthetic

SEQ ID NO: 411 - DNA, 24 bp, Artificial Sequence
  Synthetic
ggattcaccttcagtacttataac

SEQ ID NO: 412 - protein, 8 aa, Artificial Sequence
  Synthetic
GFTFSTYN

SEQ ID NO: 413 - DNA, 24 bp, Artificial Sequence
  Synthetic
attaggagtagtagtaattacata

SEQ ID NO: 414 - protein, 8 aa, Artificial Sequence
  Synthetic
IRSSSNYI

SEQ ID NO: 415 - DNA, 39 bp, Artificial Sequence; identical to SEQ ID NO: 391
  Synthetic

SEQ ID NO: 416 - protein, 13 aa, Artificial Sequence
  Synthetic
ARDGSSWYDYSDY

SEQ ID NO: 417 - DNA, 321 bp, Artificial Sequence; identical to SEQ ID NO: 393
  Synthetic

SEQ ID NO: 418 - protein, 107 aa, Artificial Sequence; identical to SEQ ID NO: 394
  Synthetic

SEQ ID NO: 419 - DNA, 18 bp, Artificial Sequence
  Synthetic
cagagtattagtagctgg

SEQ ID NO: 420 - protein, 6 aa, Artificial Sequence
  Synthetic
QSISSW

SEQ ID NO: 421 - DNA, 9 bp, Artificial Sequence
  Synthetic
aaggcgtct

SEQ ID NO: 422 - protein, 3 aa, Artificial Sequence
  Synthetic
KAS

SEQ ID NO: 423 - DNA, 27 bp, Artificial Sequence
  Synthetic
caacagtatattagttattctcggacg

SEQ ID NO: 424 - protein, 9 aa, Artificial Sequence
  Synthetic
QQYISYSRT

SEQ ID NO: 425 - DNA, 360 bp, Artificial Sequence; identical to SEQ ID NO: 401
  Synthetic

SEQ ID NO: 426 - protein, 120 aa, Artificial Sequence; identical to SEQ ID NO: 402
  Synthetic

SEQ ID NO: 427 - DNA, 321 bp, Artificial Sequence; identical to SEQ ID NO: 393
  Synthetic

SEQ ID NO: 428 - protein, 107 aa, Artificial Sequence; identical to SEQ ID NO: 394
  Synthetic

SEQ ID NO: 429 - DNA, 360 bp, Artificial Sequence; identical to SEQ ID NO: 405
  Synthetic

SEQ ID NO: 430 - protein, 120 aa, Artificial Sequence; identical to SEQ ID NO: 406
  Synthetic

SEQ ID NO: 431 - DNA, 321 bp, Artificial Sequence; identical to SEQ ID NO: 407
  Synthetic

SEQ ID NO: 432 - protein, 107 aa, Artificial Sequence; identical to SEQ ID NO: 408
  Synthetic

SEQ ID NO: 433 - DNA, 360 bp, Artificial Sequence
  Synthetic
gaggtgcagctggtggagtctgggggaggcctggtcaagccgggggggtccctgagactctcctgtacagcctctggattcaccttcagtacttataacatgaattgggtccgccaggctccagggaagggactggagtgggtctcatccattaggagtagtagtaattacatatactacgcagactcagtgaagggccgattcaccatctccagagacaacgccaagagttcactgtatctgcaaatgaacagcctgagagccgaggacacggctgtgtattactgtgcgagagatggcagcagttggtacgactactctgactactggggccagggaaccctggtcaccgtctcctca

SEQ ID NO: 434 - protein, 120 aa, Artificial Sequence
  Synthetic
EVQLVESGGGLVKPGGSLRLSCTASGFTFSTYNMNWVRQAPGKGLEWVSSIRSSSNYIYYADSVKGRFTISRDNAKSSLYLQMNSLRAEDTAVYYCARDGSSWYDYSDYWGQGTLVTVSS

SEQ ID NO: 435 - DNA, 24 bp, Artificial Sequence
  Synthetic
ggattcaccttcagtacttataac

SEQ ID NO: 436 - protein, 8 aa, Artificial Sequence
  Synthetic
GFTFSTYN

SEQ ID NO: 437 - DNA, 24 bp, Artificial Sequence
  Synthetic
attaggagtagtagtaattacata

SEQ ID NO: 438 - protein, 8 aa, Artificial Sequence
  Synthetic
IRSSSNYI

SEQ ID NO: 439 - DNA, 39 bp, Artificial Sequence; identical to SEQ ID NO: 391
  Synthetic

SEQ ID NO: 440 - protein, 13 aa, Artificial Sequence
  Synthetic
ARDGSSWYDYSDY

SEQ ID NO: 441 - DNA, 321 bp, Artificial Sequence
  Synthetic
gacatccagatgacccagtctccttccaccctgtctgcatctgtaggagacagagtcaccatcacttgccgggccagtcagagtattagtagctggttggcctggtatcaacaggtaccagggaaagcccctaaactcctgatctataaggcgtctagtttagaaaatggggtcccatcaaggttcagcggcagtggatctgggacagaattcactctcatcatcagcagcctgcagcctgatgattttgcaacttattactgccaacagtatattagttattctcggacgttcggccaagggaccaaggtggaaatcaaa

SEQ ID NO: 442 - protein, 107 aa, Artificial Sequence
  Synthetic
DIQMTQSPSTLSASVGDRVTITCRASQSISSWLAWYQQVPGKAPKLLIYKASSLENGVPSRFSGSGSGTEFTLIISSLQPDDFATYYCQQYISYSRTFGQGTKVEIK

SEQ ID NO: 443 - DNA, 18 bp, Artificial Sequence
  Synthetic
cagagtattagtagctgg

SEQ ID NO: 444 - protein, 6 aa, Artificial Sequence
  Synthetic
QSISSW

SEQ ID NO: 445 - DNA, 9 bp, Artificial Sequence
  Synthetic
aaggcgtct

SEQ ID NO: 446 - protein, 3 aa, Artificial Sequence
  Synthetic
KAS

SEQ ID NO: 447 - DNA, 27 bp, Artificial Sequence
  Synthetic
caacagtatattagttattctcggacg

SEQ ID NO: 448 - protein, 9 aa, Artificial Sequence
  Synthetic
QQYISYSRT

SEQ ID NO: 449 - DNA, 360 bp, Artificial Sequence; identical to SEQ ID NO: 433
  Synthetic

SEQ ID NO: 450 - protein, 120 aa, Artificial Sequence; identical to SEQ ID NO: 434
  Synthetic

SEQ ID NO: 451 - DNA, 321 bp, Artificial Sequence; identical to SEQ ID NO: 441
  Synthetic

SEQ ID NO: 452 - protein, 107 aa, Artificial Sequence; identical to SEQ ID NO: 442
  Synthetic

SEQ ID NO: 453 - DNA, 360 bp, Artificial Sequence
  Synthetic
gaggtgcagctggtggagtctgggggaggcctggtcaagcctggggggtccctgagactctcctgtgcagcctctggattcaccttcagtacttataacatgaactgggtccgccaggctccagggaaggggctggagtgggtctcatccattaggagtagtagtaattacatatactacgcagactcagtgaagggccgattcaccatctccagagacaacgccaagaactcactgtatctgcaaatgaacagcctgagagccgaggacacggctgtgtattactgtgcgagagatggcagcagttggtacgactactctgactactggggccagggaaccctggtcaccgtctcctca

SEQ ID NO: 454 - protein, 120 aa, Artificial Sequence; identical to SEQ ID NO: 406
  Synthetic

SEQ ID NO: 455 - DNA, 321 bp, Artificial Sequence; identical to SEQ ID NO: 407
  Synthetic

SEQ ID NO: 456 - protein, 107 aa, Artificial Sequence; identical to SEQ ID NO: 408
  Synthetic

SEQ ID NO: 457 - DNA, 360 bp, Artificial Sequence; identical to SEQ ID NO: 401
  Synthetic

SEQ ID NO: 458 - protein, 120 aa, Artificial Sequence; identical to SEQ ID NO: 402
  Synthetic

SEQ ID NO: 459 - DNA, 24 bp, Artificial Sequence
  Synthetic
ggattcaccttcagtacttataac

SEQ ID NO: 460 - protein, 8 aa, Artificial Sequence
  Synthetic
GFTFSTYN

SEQ ID NO: 461 - DNA, 24 bp, Artificial Sequence
  Synthetic
attaggagtagtagtaattacata

SEQ ID NO: 462 - protein, 8 aa, Artificial Sequence
  Synthetic
IRSSSNYI

SEQ ID NO: 463 - DNA, 39 bp, Artificial Sequence; identical to SEQ ID NO: 391
  Synthetic

SEQ ID NO: 464 - protein, 13 aa, Artificial Sequence
  Synthetic
ARDGSSWYDYSDY

SEQ ID NO: 465 - DNA, 321 bp, Artificial Sequence; identical to SEQ ID NO: 393
  Synthetic

SEQ ID NO: 466 - protein, 107 aa, Artificial Sequence; identical to SEQ ID NO: 394
  Synthetic

SEQ ID NO: 467 - DNA, 18 bp, Artificial Sequence
  Synthetic
cagagtattagtagctgg

SEQ ID NO: 468 - protein, 6 aa, Artificial Sequence
  Synthetic
QSISSW

SEQ ID NO: 469 - DNA, 9 bp, Artificial Sequence
  Synthetic
aaggcgtct

SEQ ID NO: 470 - protein, 3 aa, Artificial Sequence
  Synthetic
KAS

SEQ ID NO: 471 - DNA, 27 bp, Artificial Sequence
  Synthetic
caacagtatattagttattctcggacg

SEQ ID NO: 472 - protein, 9 aa, Artificial Sequence
  Synthetic
QQYISYSRT

SEQ ID NO: 473 - DNA, 360 bp, Artificial Sequence; identical to SEQ ID NO: 401
  Synthetic

SEQ ID NO: 474 - protein, 120 aa, Artificial Sequence; identical to SEQ ID NO: 402
  Synthetic

SEQ ID NO: 475 - DNA, 321 bp, Artificial Sequence; identical to SEQ ID NO: 393
  Synthetic

SEQ ID NO: 476 - protein, 107 aa, Artificial Sequence; identical to SEQ ID NO: 394
  Synthetic

SEQ ID NO: 477 - DNA, 360 bp, Artificial Sequence; identical to SEQ ID NO: 405
  Synthetic

SEQ ID NO: 478 - protein, 120 aa, Artificial Sequence; identical to SEQ ID NO: 406
  Synthetic

SEQ ID NO: 479 - DNA, 321 bp, Artificial Sequence; identical to SEQ ID NO: 407
  Synthetic

SEQ ID NO: 480 - protein, 107 aa, Artificial Sequence; identical to SEQ ID NO: 408
  Synthetic

SEQ ID NO: 481 - DNA, 354 bp, Artificial Sequence
  Synthetic
gaggtgcaactagtggagtctgggggaggcttggtacagcctggggggtccctgagactctcctgtgtagtctctggattcaccttcggtgactacgacatgcactgggtccgtcaagctacaggaagaggtctggagtgggtctcaggtattgctcctgctggtgacacatcctatacaggctccgtgaagggccgattcaccatctccagagagaatgccaagaactccttgcatcttcaaatgaacagcctgacaaccggggacacggctatatattattgtgctagagaggatatagcagtgcctggttttgattactggggccagggaaccctggtcaccgtctcctca

SEQ ID NO: 482 - protein, 118 aa, Artificial Sequence
  Synthetic
EVQLVESGGGLVQPGGSLRLSCVVSGFTFGDYDMHWVRQATGRGLEWVSGIAPAGDTSYTGSVKGRFTISRENAKNSLHLQMNSLTTGDTAIYYCAREDIAVPGFDYWGQGTLVTVSS

SEQ ID NO: 483 - DNA, 24 bp, Artificial Sequence
  Synthetic
ggattcaccttcggtgactacgac

SEQ ID NO: 484 - protein, 8 aa, Artificial Sequence
  Synthetic
GFTFGDYD

SEQ ID NO: 485 - DNA, 21 bp, Artificial Sequence
  Synthetic
attgctcctgctggtgacaca

SEQ ID NO: 486 - protein, 7 aa, Artificial Sequence
  Synthetic
IAPAGDT

SEQ ID NO: 487 - DNA, 36 bp, Artificial Sequence
  Synthetic
gctagagaggatatagcagtgcctggttttgattac

SEQ ID NO: 488 - protein, 12 aa, Artificial Sequence
  Synthetic
AREDIAVPGFDY

SEQ ID NO: 489 - DNA, 324 bp, Artificial Sequence
  Synthetic
gaaatagtgatgacgcagtctccagccaccctgtctgtgtctccaggggaacgaggcaccctctcctgcagggccagtcagagtgttagcagcaacttagcctggtaccagcagaaacctggccaggctcccagactcctcatctatggtgcatccacgagggccactggcttcccagccaggttcagtggcagtgggtctgggacagagttcactctcaccatcagcagcctgcagtctgaagattttgcagtttattactgtcagcagtataataagtggcctccgttcactttcggccctgggaccaaagtggatttcaaa

SEQ ID NO: 490 - protein, 108 aa, Artificial Sequence
  Synthetic
EIVMTQSPATLSVSPGERGTLSCRASQSVSSNLAWYQQKPGQAPRLLIYGASTRATGFPARFSGSGSGTEFTLTISSLQSEDFAVYYCQQYNKWPPFTFGPGTKVDFK

SEQ ID NO: 491 - DNA, 18 bp, Artificial Sequence
  Synthetic
cagagtgttagcagcaac

SEQ ID NO: 492 - protein, 6 aa, Artificial Sequence
  Synthetic
QSVSSN

SEQ ID NO: 493 - DNA, 9 bp, Artificial Sequence
  Synthetic
ggtgcatcc

SEQ ID NO: 494 - protein, 3 aa, Artificial Sequence
  Synthetic
GAS

SEQ ID NO: 495 - DNA, 30 bp, Artificial Sequence
  Synthetic
cagcagtataataagtggcctccgttcact

SEQ ID NO: 496 - protein, 10 aa, Artificial Sequence
  Synthetic
QQYNKWPPFT

SEQ ID NO: 497 - DNA, 354 bp, Artificial Sequence; identical to SEQ ID NO: 481
  Synthetic

SEQ ID NO: 498 - protein, 118 aa, Artificial Sequence; identical to SEQ ID NO: 482
  Synthetic

SEQ ID NO: 499 - DNA, 324 bp, Artificial Sequence
  Synthetic
gaaatagtgatgacgcagtctccagccaccctgtctgtgtctccaggggaacgaggcaccctctcctgcagggccagtcagagtgttagcagcaacttagcctggtaccagcagaaacctggccaggctcccagactcctcatctatggtgcatccacgagggccactggcttcccagccaggttcagtggcagtgggtctgggacagagttcactctcaccatcagcagcctgcagtctgaagattttgcagtttattactgtcagcagtataataagtggcctccgttcactttcggccctgggaccaaagtggatatcaaa

SEQ ID NO: 500 - protein, 108 aa, Artificial Sequence
  Synthetic
EIVMTQSPATLSVSPGERGTLSCRASQSVSSNLAWYQQKPGQAPRLLIYGASTRATGFPARFSGSGSGTEFTLTISSLQSEDFAVYYCQQYNKWPPFTFGPGTKVDIK

SEQ ID NO: 501 - DNA, 354 bp, Artificial Sequence
  Synthetic
gaggtgcagctggtggagtctgggggaggcttggtacagcctggggggtccctgagactctcctgtgcagcctctggattcaccttcggtgactacgacatgcactgggtccgccaagctacaggaaaaggtctggagtgggtctcagctattgctcctgctggtgacacatactatccaggctccgtgaagggccgattcaccatctccagagaaaatgccaagaactccttgtatcttcaaatgaacagcctgagagccggggacacggctgtgtattactgtgctagagaggatatagcagtgcctggttttgattactggggccaaggaaccctggtcaccgtctcctca

SEQ ID NO: 502 - protein, 118 aa, Artificial Sequence
  Synthetic
EVQLVESGGGLVQPGGSLRLSCAASGFTFGDYDMHWVRQATGKGLEWVSAIAPAGDTYYPGSVKGRFTISRENAKNSLYLQMNSLRAGDTAVYYCAREDIAVPGFDYWGQGTLVTVSS

SEQ ID NO: 503 - DNA, 324 bp, Artificial Sequence
  Synthetic
gaaatagtgatgacgcagtctccagccaccctgtctgtgtctccaggggaaagagccaccctctcctgcagggccagtcagagtgttagcagcaacttagcctggtaccagcagaaacctggccaggctcccaggctcctcatctatggtgcatccaccagggccactggtatcccagccaggttcagtggcagtgggtctgggacagagttcactctcaccatcagcagcctgcagtctgaagattttgcagtttattactgtcagcagtataataagtggcctccgttcactttcggccctgggaccaaagtggatatcaaa

SEQ ID NO: 504 - protein, 108 aa, Artificial Sequence
  Synthetic
EIVMTQSPATLSVSPGERATLSCRASQSVSSNLAWYQQKPGQAPRLLIYGASTRATGIPARFSGSGSGTEFTLTISSLQSEDFAVYYCQQYNKWPPFTFGPGTKVDIK

SEQ ID NO: 505 - DNA, 378 bp, Artificial Sequence
  Synthetic
caaattctgctggtgcaatctggacctgaggtgaaggagcctggggcctcagtgaaggtctcctgcaaggcttctggttacacctttaccaactacgctatcagctgggtgcgacaggtccctggacaagggcttgagtggatgggatgggtcagcgcttacaatggtcacacaaactatgcacatgaagtccagggcagagtcaccatgaccacagacacatccacgaccacagcctacatggagctgaggagcctgagatctgacgacacggccatgtattactgtgcgagagggggtgtagtcgtgccagttgctccccacttctacaacggtatggacgtctggggccaagggaccacggtcaccgtctcctca

SEQ ID NO: 506 - protein, 126 aa, Artificial Sequence
  Synthetic
QILLVQSGPEVKEPGASVKVSCKASGYTFTNYAISWVRQVPGQGLEWMGWVSAYNGHTNYAHEVQGRVTMTTDTSTTTAYMELRSLRSDDTAMYYCARGGVVVPVAPHFYNGMDVWGQGTTVTVSS

SEQ ID NO: 507 - DNA, 24 bp, Artificial Sequence
  Synthetic
ggttacacctttaccaactacgct

SEQ ID NO: 508 - protein, 8 aa, Artificial Sequence
  Synthetic
GYTFTNYA

SEQ ID NO: 509 - DNA, 24 bp, Artificial Sequence
  Synthetic
gtcagcgcttacaatggtcacaca

SEQ ID NO: 510 - protein, 8 aa, Artificial Sequence
  Synthetic
VSAYNGHT

SEQ ID NO: 511 - DNA, 57 bp, Artificial Sequence
  Synthetic
gcgagagggggtgtagtcgtgccagttgctccccacttctacaacggtatggacgtc

SEQ ID NO: 512 - protein, 19 aa, Artificial Sequence
  Synthetic
ARGGVVVPVAPHFYNGMDV

SEQ ID NO: 513 - DNA, 336 bp, Artificial Sequence
  Synthetic
gatattgtgatgactcagtttccactctccctgcccgtcacccctggagagccggcctccatctcctgcaggtctagtcagagcctcctgcatattaatgaatacaactatttggattggtacctaaagaagccagggcagtctccacagctcctgatctatttgggttttaatcgggcctccggggtccctgacaggttcagtggcagtggatcaggcacagattttacactgaaaatcagcagagtggaggctgaggatgttggggtctattactgcatgcaagctcttcaaactccgtggacgttaggccaagggaccaaggtggaaatcaaa

SEQ ID NO: 514 - protein, 112 aa, Artificial Sequence
  Synthetic
DIVMTQFPLSLPVTPGEPASISCRSSQSLLHINEYNYLDWYLKKPGQSPQLLIYLGFNRASGVPDRFSGSGSGTDFTLKISRVEAEDVGVYYCMQALQTPWTLGQGTKVEIK

SEQ ID NO: 515 - DNA, 33 bp, Artificial Sequence
  Synthetic
cagagcctcctgcatattaatgaatacaactat

SEQ ID NO: 516 - protein, 11 aa, Artificial Sequence
  Synthetic
QSLLHINEYNY

SEQ ID NO: 517 - DNA, 9 bp, Artificial Sequence
  Synthetic
ttgggtttt

SEQ ID NO: 518 - protein, 3 aa, Artificial Sequence
  Synthetic
LGF

SEQ ID NO: 519 - DNA, 27 bp, Artificial Sequence
  Synthetic
atgcaagctcttcaaactccgtggacg

SEQ ID NO: 520 - protein, 9 aa, Artificial Sequence
  Synthetic
MQALQTPWT

SEQ ID NO: 521 - DNA, 378 bp, Artificial Sequence
  Synthetic
caggttcagctggtgcagtctggacctgaggtgaaggagcctggggcctcagtgaaggtctcctgcaaggcttctggttacacctttaccaactacgctatcagctgggtgcgacaggtccctggacaagggcttgagtggatgggatgggtcagcgcttacaatggtcacacaaactatgcacatgaagtccagggcagagtcaccatgaccacagacacatccacgaccacagcctacatggagctgaggagcctgagatctgacgacacggccatgtattactgtgcgagagggggtgtagtcgtgccagttgctccccacttctacaacggtatggacgtctggggccaagggaccacggtcaccgtctcctca

SEQ ID NO: 522 - protein, 126 aa, Artificial Sequence
  Synthetic
QVQLVQSGPEVKEPGASVKVSCKASGYTFTNYAISWVRQVPGQGLEWMGWVSAYNGHTNYAHEVQGRVTMTTDTSTTTAYMELRSLRSDDTAMYYCARGGVVVPVAPHFYNGMDVWGQGTTVTVSS

SEQ ID NO: 523 - DNA, 336 bp, Artificial Sequence
  Synthetic
gatattgtgatgactcagtctccactctccctgcccgtcacccctggagagccggcctccatctcctgcaggtctagtcagagcctcctgcatattaatgaatacaactatttggattggtacctaaagaagccagggcagtctccacagctcctgatctatttgggttttaatcgggcctccggggtccctgacaggttcagtggcagtggatcaggcacagattttacactgaaaatcagcagagtggaggctgaggatgttggggtctattactgcatgcaagctcttcaaactccgtggacgttaggccaagggaccaaggtggaaatcaaa

SEQ ID NO: 524 - protein, 112 aa, Artificial Sequence
  Synthetic
DIVMTQSPLSLPVTPGEPASISCRSSQSLLHINEYNYLDWYLKKPGQSPQLLIYLGFNRASGVPDRFSGSGSGTDFTLKISRVEAEDVGVYYCMQALQTPWTLGQGTKVEIK

SEQ ID NO: 525 - DNA, 378 bp, Artificial Sequence
  Synthetic
caggttcagctggtgcagtctggagctgaggtgaagaagcctggggcctcagtgaaggtctcctgcaaggcttctggttacacctttaccaactacgctatcagctgggtgcgacaggcccctggacaagggcttgagtggatgggatgggtcagcgcttacaatggtcacacaaactatgcacagaagctccagggcagagtcaccatgaccacagacacatccacgagcacagcctacatggagctgaggagcctgagatctgacgacacggccgtgtattactgtgcgagagggggtgtagtcgtgccagttgctccccacttctacaacggtatggacgtctgggggcaagggaccacggtcaccgtctcctca

SEQ ID NO: 526 - protein, 126 aa, Artificial Sequence
  Synthetic
QVQLVQSGAEVKKPGASVKVSCKASGYTFTNYAISWVRQAPGQGLEWMGWVSAYNGHTNYAQKLQGRVTMTTDTSTSTAYMELRSLRSDDTAVYYCARGGVVVPVAPHFYNGMDVWGQGTTVTVSS

SEQ ID NO: 527 - DNA, 336 bp, Artificial Sequence
  Synthetic
gatattgtgatgactcagtctccactctccctgcccgtcacccctggagagccggcctccatctcctgcaggtctagtcagagcctcctgcatattaatgaatacaactatttggattggtacctgcagaagccagggcagtctccacagctcctgatctatttgggttctaatcgggcctccggggtccctgacaggttcagtggcagtggatcaggcacagattttacactgaaaatcagcagagtggaggctgaggatgttggggtttattactgcatgcaagctcttcaaactccgtggacgttcggccaagggaccaaggtggaaatcaaa

SEQ ID NO: 528 - protein, 112 aa, Artificial Sequence
  Synthetic
DIVMTQSPLSLPVTPGEPASISCRSSQSLLHINEYNYLDWYLQKPGQSPQLLIYLGSNRASGVPDRFSGSGSGTDFTLKISRVEAEDVGVYYCMQALQTPWTFGQGTKVEIK

SEQ ID NO: 529 - DNA, 351 bp, Artificial Sequence
  Synthetic
gaggtgcagctggtggagtctgggggaggcttggtacagcctggggggtccctgagactctcctgtgcagcctctggattcaccctaagtagctacgacatgcactgggtccgccaagcaacaggaaaaggtctggagtgggtctcagctattggcagtactggtgacacatactatacaggctccgtgatgggccgattcaccatctccagagacgctgccaaaaactccttctatcttgaaatgaacagcctgagagtcggggacacggctgtatattactgtgcaagagagggaataagaacaccctatgattattggggccagggagcccgggtcaccgtctcctca

SEQ ID NO: 530 - protein, 117 aa, Artificial Sequence
  Synthetic
EVQLVESGGGLVQPGGSLRLSCAASGFTLSSYDMHWVRQATGKGLEWVSAIGSTGDTYYTGSVMGRFTISRDAAKNSFYLEMNSLRVGDTAVYYCAREGIRTPYDYWGQGARVTVSS

SEQ ID NO: 531 - DNA, 24 bp, Artificial Sequence
  Synthetic
ggattcaccctaagtagctacgac

SEQ ID NO: 532 - protein, 8 aa, Artificial Sequence
  Synthetic
GFTLSSYD

SEQ ID NO: 533 - DNA, 21 bp, Artificial Sequence
  Synthetic
attggcagtactggtgacaca

SEQ ID NO: 534 - protein, 7 aa, Artificial Sequence
  Synthetic
IGSTGDT

SEQ ID NO: 535 - DNA, 33 bp, Artificial Sequence
  Synthetic
gcaagagagggaataagaacaccctatgattat

SEQ ID NO: 536 - protein, 11 aa, Artificial Sequence
  Synthetic
AREGIRTPYDY

SEQ ID NO: 537 - DNA, 324 bp, Artificial Sequence
  Synthetic
gaaatagtgatgacgcagtctccagccaccctgtctgtgtctccaggggaaagagccaccctctcctgcagggccagtcagagtgttagcagcaatgtagcctggtaccagcagaaacctggccaggctcccaggctcctcatctatggtgcatccaccagggccactggtatcccagccaggttcagtggcagtgggtctgggacagaattcactctcaccatcagcagcctgcagtctgaagattttgcagtttattactgtcagcagtataataattggcctccattcactttcggccctgggaccaaagtggatatcaaa

SEQ ID NO: 538 - protein, 108 aa, Artificial Sequence
  Synthetic
EIVMTQSPATLSVSPGERATLSCRASQSVSSNVAWYQQKPGQAPRLLIYGASTRATGIPARFSGSGSGTEFTLTISSLQSEDFAVYYCQQYNNWPPFTFGPGTKVDIK

SEQ ID NO: 539 - DNA, 18 bp, Artificial Sequence
  Synthetic
cagagtgttagcagcaat

SEQ ID NO: 540 - protein, 6 aa, Artificial Sequence
  Synthetic
QSVSSN

SEQ ID NO: 541 - DNA, 9 bp, Artificial Sequence
  Synthetic
ggtgcatcc

SEQ ID NO: 542 - protein, 3 aa, Artificial Sequence
  Synthetic
GAS

SEQ ID NO: 543 - DNA, 30 bp, Artificial Sequence
  Synthetic
cagcagtataataattggcctccattcact

SEQ ID NO: 544 - protein, 10 aa, Artificial Sequence
  Synthetic
QQYNNWPPFT

SEQ ID NO: 545 - DNA, 351 bp, Artificial Sequence
  Synthetic
gaggtgcagctggtggagtctgggggaggcttggtacagcctggggggtccctgagactctcctgtgcagcctctggattcaccctaagtagctacgacatgcactgggtccgccaagcaacaggaaaaggtctggagtgggtctcagctattggcagtactggtgacacatactatacaggctccgtgatgggccgattcaccatctccagagacgctgccaaaaactccttctatcttgaaatgaacagcctgagagtcggggacacggctgtatattactgtgcaagagagggaataagaacaccctatgattattggggccagggaaccctggtcaccgtctcctca

SEQ ID NO: 546 - protein, 117 aa, Artificial Sequence
  Synthetic
EVQLVESGGGLVQPGGSLRLSCAASGFTLSSYDMHWVRQATGKGLEWVSAIGSTGDTYYTGSVMGRFTISRDAAKNSFYLEMNSLRVGDTAVYYCAREGIRTPYDYWGQGTLVTVSS

SEQ ID NO: 547 - DNA, 324 bp, Artificial Sequence; identical to SEQ ID NO: 537
  Synthetic

SEQ ID NO: 548 - protein, 108 aa, Artificial Sequence; identical to SEQ ID NO: 538
  Synthetic

SEQ ID NO: 549 - DNA, 351 bp, Artificial Sequence
  Synthetic
gaggtgcagctggtggagtctgggggaggcttggtacagcctggggggtccctgagactctcctgtgcagcctctggattcaccctaagtagctacgacatgcactgggtccgccaagctacaggaaaaggtctggagtgggtctcagctattggcagtactggtgacacatactatccaggctccgtgaagggccgattcaccatctccagagaaaatgccaagaactccttgtatcttcaaatgaacagcctgagagccggggacacggctgtgtattactgtgcaagagagggaataagaacaccctatgattattggggccaaggaaccctggtcaccgtctcctca

SEQ ID NO: 550 - protein, 117 aa, Artificial Sequence
  Synthetic
EVQLVESGGGLVQPGGSLRLSCAASGFTLSSYDMHWVRQATGKGLEWVSAIGSTGDTYYPGSVKGRFTISRENAKNSLYLQMNSLRAGDTAVYYCAREGIRTPYDYWGQGTLVTVSS

SEQ ID NO: 551 - DNA, 324 bp, Artificial Sequence
  Synthetic
gaaatagtgatgacgcagtctccagccaccctgtctgtgtctccaggggaaagagccaccctctcctgcagggccagtcagagtgttagcagcaatttagcctggtaccagcagaaacctggccaggctcccaggctcctcatctatggtgcatccaccagggccactggtatcccagccaggttcagtggcagtgggtctgggacagagttcactctcaccatcagcagcctgcagtctgaagattttgcagtttattactgtcagcagtataataattggcctccattcactttcggccctgggaccaaagtggatatcaaa

SEQ ID NO: 552 - protein, 108 aa, Artificial Sequence; identical to SEQ ID NO: 24
  Synthetic

SEQ ID NO: 553 - DNA, 351 bp, Artificial Sequence; identical to SEQ ID NO: 529
  Synthetic

SEQ ID NO: 554 - protein, 117 aa, Artificial Sequence; identical to SEQ ID NO: 530
  Synthetic

SEQ ID NO: 555 - DNA, 24 bp, Artificial Sequence
  Synthetic
ggattcaccctaagtagctacgac

SEQ ID NO: 556 - protein, 8 aa, Artificial Sequence
  Synthetic
GFTLSSYD

SEQ ID NO: 557 - DNA, 21 bp, Artificial Sequence
  Synthetic
attggcagtactggtgacaca

SEQ ID NO: 558 - protein, 7 aa, Artificial Sequence
  Synthetic
IGSTGDT

SEQ ID NO: 559 - DNA, 33 bp, Artificial Sequence; identical to SEQ ID NO: 535
  Synthetic

SEQ ID NO: 560 - protein, 11 aa, Artificial Sequence
  Synthetic
AREGIRTPYDY

SEQ ID NO: 561 - DNA, 324 bp, Artificial Sequence; identical to SEQ ID NO: 537
  Synthetic

SEQ ID NO: 562 - protein, 108 aa, Artificial Sequence; identical to SEQ ID NO: 538
  Synthetic

SEQ ID NO: 563 - DNA, 18 bp, Artificial Sequence
  Synthetic
cagagtgttagcagcaat

SEQ ID NO: 564 - protein, 6 aa, Artificial Sequence
  Synthetic
QSVSSN

SEQ ID NO: 565 - DNA, 9 bp, Artificial Sequence
  Synthetic
ggtgcatcc

SEQ ID NO: 566 - protein, 3 aa, Artificial Sequence
  Synthetic
GAS

SEQ ID NO: 567 - DNA, 30 bp, Artificial Sequence; identical to SEQ ID NO: 543
  Synthetic

SEQ ID NO: 568 - protein, 10 aa, Artificial Sequence
  Synthetic
QQYNNWPPFT

SEQ ID NO: 569 - DNA, 351 bp, Artificial Sequence; identical to SEQ ID NO: 545
  Synthetic

SEQ ID NO: 570 - protein, 117 aa, Artificial Sequence; identical to SEQ ID NO: 546
  Synthetic

SEQ ID NO: 571 - DNA, 324 bp, Artificial Sequence; identical to SEQ ID NO: 537
  Synthetic

SEQ ID NO: 572 - protein, 108 aa, Artificial Sequence; identical to SEQ ID NO: 538
  Synthetic

SEQ ID NO: 573 - DNA, 351 bp, Artificial Sequence; identical to SEQ ID NO: 549
  Synthetic

SEQ ID NO: 574 - protein, 117 aa, Artificial Sequence; identical to SEQ ID NO: 550
  Synthetic

SEQ ID NO: 575 - DNA, 324 bp, Artificial Sequence; identical to SEQ ID NO: 551
  Synthetic

SEQ ID NO: 576 - protein, 108 aa, Artificial Sequence; identical to SEQ ID NO: 24
  Synthetic

SEQ ID NO: 577 - DNA, 363 bp, Artificial Sequence
  Synthetic
gaagtgcagctggtggagtctgggggaggcttggtacagcctggcaggtccctgagactctcctgtgcagcctctggattcacctttgatgattatgccatgcactgggtccggcaagctccagggaagggcctggagtgggtctcaggtattaattggaacagtggtagcataggctatgcggactctgtgaagggccgattcaccatctccagagacaacgccaagcactccctgtatctgcaaatgaacagtctgagacctgaggacacggccttgtattactgtgtaaaagaggtgactacgggatactactacggtatggacgtctggggccaagggaccacggtcaccgtctcctca

SEQ ID NO: 578 - protein, 121 aa, Artificial Sequence
  Synthetic
EVQLVESGGGLVQPGRSLRLSCAASGFTFDDYAMHWVRQAPGKGLEWVSGINWNSGSIGYADSVKGRFTISRDNAKHSLYLQMNSLRPEDTALYYCVKEVTTGYYYGMDVWGQGTTVTVSS

SEQ ID NO: 579 - DNA, 24 bp, Artificial Sequence
  Synthetic
ggattcacctttgatgattatgcc

SEQ ID NO: 580 - protein, 8 aa, Artificial Sequence
  Synthetic
GFTFDDYA

SEQ ID NO: 581 - DNA, 24 bp, Artificial Sequence
  Synthetic
attaattggaacagtggtagcata

SEQ ID NO: 582 - protein, 8 aa, Artificial Sequence
  Synthetic
INWNSGSI

SEQ ID NO: 583 - DNA, 42 bp, Artificial Sequence
  Synthetic
gtaaaagaggtgactacgggatactactacggtatggacgtc

SEQ ID NO: 584 - protein, 14 aa, Artificial Sequence
  Synthetic
VKEVTTGYYYGMDV

SEQ ID NO: 585 - DNA, 321 bp, Artificial Sequence
  Synthetic
gacatccagttgacccagtctccatccttcctgtctgcatctgtaggagacagagtcaccatcacttgctgggccagtcagggcattagcagttatttagcctggtatcagaaaaaaccagggaaagcccctaacctcctgatctatgatgcatccactttgcaaagtggggtcccatcaaggttcagcggcagtggatctgggacagaattcactctcacactcagcagcctgcagcctgaagattttgcaacttattactgtcaacagcttaatatttacccattcactttcggccctgggaccaaagtggatatcaaa

SEQ ID NO: 586 - protein, 107 aa, Artificial Sequence
  Synthetic
DIQLTQSPSFLSASVGDRVTITCWASQGISSYLAWYQKKPGKAPNLLIYDASTLQSGVPSRFSGSGSGTEFTLTLSSLQPEDFATYYCQQLNIYPFTFGPGTKVDIK

SEQ ID NO: 587 - DNA, 18 bp, Artificial Sequence
  Synthetic
cagggcattagcagttat

SEQ ID NO: 588 - protein, 6 aa, Artificial Sequence
  Synthetic
QGISSY

SEQ ID NO: 589 - DNA, 9 bp, Artificial Sequence
  Synthetic
gatgcatcc

SEQ ID NO: 590 - protein, 3 aa, Artificial Sequence
  Synthetic
DAS

SEQ ID NO: 591 - DNA, 27 bp, Artificial Sequence
  Synthetic
caacagcttaatatttacccattcact

SEQ ID NO: 592 - protein, 9 aa, Artificial Sequence
  Synthetic
QQLNIYPFT

SEQ ID NO: 593 - DNA, 363 bp, Artificial Sequence; identical to SEQ ID NO: 577
  Synthetic

SEQ ID NO: 594 - protein, 121 aa, Artificial Sequence; identical to SEQ ID NO: 578
  Synthetic

SEQ ID NO: 595 - DNA, 321 bp, Artificial Sequence; identical to SEQ ID NO: 585
  Synthetic

SEQ ID NO: 596 - protein, 107 aa, Artificial Sequence; identical to SEQ ID NO: 586
  Synthetic

SEQ ID NO: 597 - DNA, 363 bp, Artificial Sequence
  Synthetic
gaagtgcagctggtggagtctgggggaggcttggtacagcctggcaggtccctgagactctcctgtgcagcctctggattcacctttgatgattatgccatgcactgggtccggcaagctccagggaagggcctggagtgggtctcaggtattaattggaacagtggtagcataggctatgcggactctgtgaagggccgattcaccatctccagagacaacgccaagaactccctgtatctgcaaatgaacagtctgagagctgaggacacggccttgtattactgtgtaaaagaggtgactacgggatactactacggtatggacgtctgggggcaagggaccacggtcaccgtctcctca

SEQ ID NO: 598 - protein, 121 aa, Artificial Sequence
  Synthetic
EVQLVESGGGLVQPGRSLRLSCAASGFTFDDYAMHWVRQAPGKGLEWVSGINWNSGSIGYADSVKGRFTISRDNAKNSLYLQMNSLRAEDTALYYCVKEVTTGYYYGMDVWGQGTTVTVSS

SEQ ID NO: 599 - DNA, 321 bp, Artificial Sequence
  Synthetic
gacatccagttgacccagtctccatccttcctgtctgcatctgtaggagacagagtcaccatcacttgccgggccagtcagggcattagcagttatttagcctggtatcagcaaaaaccagggaaagcccctaagctcctgatctatgatgcatccactttgcaaagtggggtcccatcaaggttcagcggcagtggatctgggacagaattcactctcacaatcagcagcctgcagcctgaagattttgcaacttattactgtcaacagcttaatatttacccattcactttcggccctgggaccaaagtggatatcaaa

SEQ ID NO: 600 - protein, 107 aa, Artificial Sequence
  Synthetic
DIQLTQSPSFLSASVGDRVTITCRASQGISSYLAWYQQKPGKAPKLLIYDASTLQSGVPSRFSGSGSGTEFTLTISSLQPEDFATYYCQQLNIYPFTFGPGTKVDIK

SEQ ID NO: 601 - DNA, 366 bp, Artificial Sequence
  Synthetic
gaggtgcagttgttggagtctgggggaggcttggtacagcctggggggtccctgagactctcctgtgcagcctctggattcacgtttagtagctatgccatgaactgggtccgccaggctccagggaaggggctggattgggtctcaggtatcagtggtaatggtggtagcacctactacgcagactccgtgaagggccggttcaccatctccagagacatttccaagaacacgctgtatgtgcaaatgcacagcctgagagtcgaggacacggccgtttactactgtgcgaaagcccgttattacgatttttggggggggaatttcgatctctggggccgtggcacccaggtcactgtctcctca

SEQ ID NO: 602 - protein, 122 aa, Artificial Sequence
  Synthetic
EVQLLESGGGLVQPGGSLRLSCAASGFTFSSYAMNWVRQAPGKGLDWVSGISGNGGSTYYADSVKGRFTISRDISKNTLYVQMHSLRVEDTAVYYCAKARYYDFWGGNFDLWGRGTQVTVSS

SEQ ID NO: 603 - DNA, 24 bp, Artificial Sequence
  Synthetic
ggattcacgtttagtagctatgcc

SEQ ID NO: 604 - protein, 8 aa, Artificial Sequence
  Synthetic
GFTFSSYA

SEQ ID NO: 605 - DNA, 24 bp, Artificial Sequence
  Synthetic
atcagtggtaatggtggtagcacc

SEQ ID NO: 606 - protein, 8 aa, Artificial Sequence
  Synthetic
ISGNGGST

SEQ ID NO: 607 - DNA, 45 bp, Artificial Sequence
  Synthetic
gcgaaagcccgttattacgatttttggggggggaatttcgatctc

SEQ ID NO: 608 - protein, 15 aa, Artificial Sequence
  Synthetic
AKARYYDFWGGNFDL

SEQ ID NO: 609 - DNA, 324 bp, Artificial Sequence
  Synthetic
gaaattgtgttgacgcagtctccaggcaccctgtctttgtctccaggggaaagagccaccctctcctgcagggccagtcagagtgttagcatcaggtacttagcctggtatcagcagaaacctggccaggctcccaggctcctcatctatggtgcatccagcagggccactggcatcccagacaggttcagtgtcagtgtgtctgggacagacttcactctcaccatcactagactggagcctgaagattttgcagtctattactgtcagcaatatggtagttcaccgctcactttcggcggagggaccaaggtggagatcaaa

SEQ ID NO: 610 - protein, 108 aa, Artificial Sequence
  Synthetic
EIVLTQSPGTLSLSPGERATLSCRASQSVSIRYLAWYQQKPGQAPRLLIYGASSRATGIPDRFSVSVSGTDFTLTITRLEPEDFAVYYCQQYGSSPLTFGGGTKVEIK

SEQ ID NO: 611 - DNA, 21 bp, Artificial Sequence
  Synthetic
cagagtgttagcatcaggtac

SEQ ID NO: 612 - protein, 7 aa, Artificial Sequence
  Synthetic
QSVSIRY

SEQ ID NO: 613 - DNA, 9 bp, Artificial Sequence
  Synthetic
ggtgcatcc

SEQ ID NO: 614 - protein, 3 aa, Artificial Sequence
  Synthetic
GAS

SEQ ID NO: 615 - DNA, 27 bp, Artificial Sequence
  Synthetic
cagcaatatggtagttcaccgctcact

SEQ ID NO: 616 - protein, 9 aa, Artificial Sequence
  Synthetic
QQYGSSPLT

SEQ ID NO: 617 - DNA, 366 bp, Artificial Sequence
  Synthetic
gaggtgcagttgttggagtctgggggaggcttggtacagcctggggggtccctgagactctcctgtgcagcctctggattcacgtttagtagctatgccatgaactgggtccgccaggctccagggaaggggctggattgggtctcaggtatcagtggtaatggtggtagcacctactacgcagactccgtgaagggccggttcaccatctccagagacatttccaagaacacgctgtatgtgcaaatgcacagcctgagagtcgaggacacggccgtttactactgtgcgaaagcccgttattacgatttttggggggggaatttcgatctctggggccgtggcaccctggtcactgtctcctca

SEQ ID NO: 618 - protein, 122 aa, Artificial Sequence
  Synthetic
EVQLLESGGGLVQPGGSLRLSCAASGFTFSSYAMNWVRQAPGKGLDWVSGISGNGGSTYYADSVKGRFTISRDISKNTLYVQMHSLRVEDTAVYYCAKARYYDFWGGNFDLWGRGTLVTVSS

SEQ ID NO: 619 - DNA, 324 bp, Artificial Sequence; identical to SEQ ID NO: 609
  Synthetic

SEQ ID NO: 620 - protein, 108 aa, Artificial Sequence; identical to SEQ ID NO: 610
  Synthetic

SEQ ID NO: 621 - DNA, 366 bp, Artificial Sequence
  Synthetic
gaggtgcagctgttggagtctgggggaggcttggtacagcctggggggtccctgagactctcctgtgcagcctctggattcacgtttagtagctatgccatgagctgggtccgccaggctccagggaaggggctggagtgggtctcagctatcagtggtaatggtggtagcacctactacgcagactccgtgaagggccggttcaccatctccagagacaattccaagaacacgctgtatctgcaaatgaacagcctgagagccgaggacacggccgtatattactgtgcgaaagcccgttattacgatttttggggggggaatttcgatctctggggccgtggcaccctggtcactgtctcctca

SEQ ID NO: 622 - protein, 122 aa, Artificial Sequence
  Synthetic
EVQLLESGGGLVQPGGSLRLSCAASGFTFSSYAMSWVRQAPGKGLEWVSAISGNGGSTYYADSVKGRFTISRDNSKNTLYLQMNSLRAEDTAVYYCAKARYYDFWGGNFDLWGRGTLVTVSS

SEQ ID NO: 623 - DNA, 324 bp, Artificial Sequence
  Synthetic
gaaattgtgttgacgcagtctccaggcaccctgtctttgtctccaggggaaagagccaccctctcctgcagggccagtcagagtgttagcatcaggtacttagcctggtaccagcagaaacctggccaggctcccaggctcctcatctatggtgcatccagcagggccactggcatcccagacaggttcagtggcagtgggtctgggacagacttcactctcaccatcagcagactggagcctgaagattttgcagtgtattactgtcagcaatatggtagttcaccgctcactttcggcggagggaccaaggtggagatcaaa

SEQ ID NO: 624 - protein, 108 aa, Artificial Sequence
  Synthetic
EIVLTQSPGTLSLSPGERATLSCRASQSVSIRYLAWYQQKPGQAPRLLIYGASSRATGIPDRFSGSGSGTDFTLTISRLEPEDFAVYYCQQYGSSPLTFGGGTKVEIK

SEQ ID NO: 625 - DNA, 381 bp, Artificial Sequence
  Synthetic
caggttcagctggtgcagtctggacctgaggtgaagaaccctggggcctcagtgaaggtctcctgcaaggcttctggttacacctttaccacctatggtatcagttgggtacgacaggcccctggacaagggcttgagtggatgggatggatcagcggttacaatggtaaaacaaacgatgcacagaagttccaggacagagtcgccatgaccacagacacatccacgagcacagcctacatggagctgaggagcctgagatctgacgacacggccatttattactgttcgagagatcgtttagtagtaccacctgccctttattattcctactacgttatggacgtctggggccaagggaccacggtcaccgtctcctca

SEQ ID NO: 626 - protein, 127 aa, Artificial Sequence
  Synthetic
QVQLVQSGPEVKNPGASVKVSCKASGYTFTTYGISWVRQAPGQGLEWMGWISGYNGKTNDAQKFQDRVAMTTDTSTSTAYMELRSLRSDDTAIYYCSRDRLVVPPALYYSYYVMDVWGQGTTVTVSS

SEQ ID NO: 627 - DNA, 24 bp, Artificial Sequence
  Synthetic
ggttacacctttaccacctatggt

SEQ ID NO: 628 - protein, 8 aa, Artificial Sequence
  Synthetic
GYTFTTYG

SEQ ID NO: 629 - DNA, 24 bp, Artificial Sequence
  Synthetic
atcagcggttacaatggtaaaaca

SEQ ID NO: 630 - protein, 8 aa, Artificial Sequence
  Synthetic
ISGYNGKT

SEQ ID NO: 631 - DNA, 60 bp, Artificial Sequence
  Synthetic
tcgagagatcgtttagtagtaccacctgccctttattattcctactacgttatggacgtc

SEQ ID NO: 632 - protein, 20 aa, Artificial Sequence
  Synthetic
SRDRLVVPPALYYSYYVMDV

SEQ ID NO: 633 - DNA, 336 bp, Artificial Sequence
  Synthetic
gatgttgtgatgactcagtctccactctccctgcccgtcacccttggacagccggcctccatctcctgcaggtctagtcaaagcctcgtatacagtgatggaaacacctacttgaattggtttcagcagaggccaggtcaatctccaaggcgcctaatttataaggtttctaaccgggactctggggtcccagacagattcagcggcagtgggtcaggcactgatttcacactgaaaatcagcagggtggaggctgaggatgttggggtttattactgcatgcaaggtacacactggccgtacacttttggccaggggaccaagctggagatcaaa

SEQ ID NO: 634 - protein, 112 aa, Artificial Sequence; identical to SEQ ID NO: 336
  Synthetic

SEQ ID NO: 635 - DNA, 33 bp, Artificial Sequence; identical to SEQ ID NO: 323
  Synthetic

SEQ ID NO: 636 - protein, 11 aa, Artificial Sequence
  Synthetic
QSLVYSDGNTY

SEQ ID NO: 637 - DNA, 9 bp, Artificial Sequence
  Synthetic
aaggtttct

SEQ ID NO: 638 - protein, 3 aa, Artificial Sequence
  Synthetic
KVS

SEQ ID NO: 639 - DNA, 27 bp, Artificial Sequence
  Synthetic
atgcaaggtacacactggccgtacact

SEQ ID NO: 640 - protein, 9 aa, Artificial Sequence
  Synthetic
MQGTHWPYT

SEQ ID NO: 641 - DNA, 381 bp, Artificial Sequence; identical to SEQ ID NO: 625
  Synthetic

SEQ ID NO: 642 - protein, 127 aa, Artificial Sequence; identical to SEQ ID NO: 626
  Synthetic

SEQ ID NO: 643 - DNA, 336 bp, Artificial Sequence; identical to SEQ ID NO: 633
  Synthetic

SEQ ID NO: 644 - protein, 112 aa, Artificial Sequence; identical to SEQ ID NO: 336
  Synthetic

SEQ ID NO: 645 - DNA, 381 bp, Artificial Sequence
  Synthetic
caggttcagctggtgcagtctggagctgaggtgaagaagcctggggcctcagtgaaggtctcctgcaaggcttctggttacacctttaccacctatggtatcagctgggtgcgacaggcccctggacaagggcttgagtggatgggatggatcagcggttacaatggtaaaacaaactatgcacagaagctccagggcagagtcaccatgaccacagacacatccacgagcacagcctacatggagctgaggagcctgagatctgacgacacggccgtgtattactgttcgagagatcgtttagtagtaccacctgccctttattattcctactacgttatggacgtctgggggcaagggaccacggtcaccgtctcctca

SEQ ID NO: 646 - protein, 127 aa, Artificial Sequence
  Synthetic
QVQLVQSGAEVKKPGASVKVSCKASGYTFTTYGISWVRQAPGQGLEWMGWISGYNGKTNYAQKLQGRVTMTTDTSTSTAYMELRSLRSDDTAVYYCSRDRLVVPPALYYSYYVMDVWGQGTTVTVSS

SEQ ID NO: 647 - DNA, 336 bp, Artificial Sequence; identical to SEQ ID NO: 335
  Synthetic

SEQ ID NO: 648 - protein, 112 aa, Artificial Sequence; identical to SEQ ID NO: 336
  Synthetic

SEQ ID NO: 649 - DNA, 381 bp, Artificial Sequence
  Synthetic
caggttcagctggtgcagtctggacctgaggtgaagaaccctggggcctcagtgaaggtctcctgcaaggcttctggttacacctttaccacctatggtatcagttgggtacgacaggcccctggacaagggcttgagtggatgggatggatcagcggttacaatggtaaaacaaacgatgcacagaagttccaggacagagtcgccatgaccacagacacatccacgagcacagcctacatggagctgaggagcctgagatctgacgacacggccatttattactgttcgagagatcgtttagtagtaccacctgcccttaattattactactacgttatggacgtctggggccaagggaccacggtcaccgtctcctca

SEQ ID NO: 650 - protein, 127 aa, Artificial Sequence
  Synthetic
QVQLVQSGPEVKNPGASVKVSCKASGYTFTTYGISWVRQAPGQGLEWMGWISGYNGKTNDAQKFQDRVAMTTDTSTSTAYMELRSLRSDDTAIYYCSRDRLVVPPALNYYYYVMDVWGQGTTVTVSS

SEQ ID NO: 651 - DNA, 24 bp, Artificial Sequence
  Synthetic
ggttacacctttaccacctatggt

SEQ ID NO: 652 - protein, 8 aa, Artificial Sequence
  Synthetic
GYTFTTYG

SEQ ID NO: 653 - DNA, 24 bp, Artificial Sequence
  Synthetic
atcagcggttacaatggtaaaaca

SEQ ID NO: 654 - protein, 8 aa, Artificial Sequence
  Synthetic
ISGYNGKT

SEQ ID NO: 655 - DNA, 60 bp, Artificial Sequence
  Synthetic
tcgagagatcgtttagtagtaccacctgcccttaattattactactacgttatggacgtc

SEQ ID NO: 656 - protein, 20 aa, Artificial Sequence
  Synthetic
SRDRLVVPPALNYYYYVMDV

SEQ ID NO: 657 - DNA, 336 bp, Artificial Sequence; identical to SEQ ID NO: 633
  Synthetic

SEQ ID NO: 658 - protein, 112 aa, Artificial Sequence; identical to SEQ ID NO: 336
  Synthetic

SEQ ID NO: 659 - DNA, 33 bp, Artificial Sequence; identical to SEQ ID NO: 323
  Synthetic

SEQ ID NO: 660 - protein, 11 aa, Artificial Sequence
  Synthetic
QSLVYSDGNTY

SEQ ID NO: 661 - DNA, 9 bp, Artificial Sequence
  Synthetic
aaggtttct

SEQ ID NO: 662 - protein, 3 aa, Artificial Sequence
  Synthetic
KVS

SEQ ID NO: 663 - DNA, 27 bp, Artificial Sequence
  Synthetic
atgcaaggtacacactggccgtacact

SEQ ID NO: 664 - protein, 9 aa, Artificial Sequence
  Synthetic
MQGTHWPYT

SEQ ID NO: 665 - DNA, 381 bp, Artificial Sequence; identical to SEQ ID NO: 649
  Synthetic

SEQ ID NO: 666 - protein, 127 aa, Artificial Sequence; identical to SEQ ID NO: 650
  Synthetic

SEQ ID NO: 667 - DNA, 336 bp, Artificial Sequence; identical to SEQ ID NO: 633
  Synthetic

SEQ ID NO: 668 - protein, 112 aa, Artificial Sequence; identical to SEQ ID NO: 336
  Synthetic

SEQ ID NO: 669 - DNA, 381 bp, Artificial Sequence
  Synthetic
caggttcagctggtgcagtctggagctgaggtgaagaagcctggggcctcagtgaaggtctcctgcaaggcttctggttacacctttaccacctatggtatcagctgggtgcgacaggcccctggacaagggcttgagtggatgggatggatcagcggttacaatggtaaaacaaactatgcacagaagctccagggcagagtcaccatgaccacagacacatccacgagcacagcctacatggagctgaggagcctgagatctgacgacacggccgtgtattactgttcgagagatcgtttagtagtaccacctgcccttaattattactactacgttatggacgtctgggggcaagggaccacggtcaccgtctcctca

SEQ ID NO: 670 - protein, 127 aa, Artificial Sequence
  Synthetic
QVQLVQSGAEVKKPGASVKVSCKASGYTFTTYGISWVRQAPGQGLEWMGWISGYNGKTNYAQKLQGRVTMTTDTSTSTAYMELRSLRSDDTAVYYCSRDRLVVPPALNYYYYVMDVWGQGTTVTVSS

SEQ ID NO: 671 - DNA, 336 bp, Artificial Sequence; identical to SEQ ID NO: 335
  Synthetic

SEQ ID NO: 672 - protein, 112 aa, Artificial Sequence; identical to SEQ ID NO: 336
  Synthetic

SEQ ID NO: 673 - DNA, 381 bp, Artificial Sequence
  Synthetic
caggttcagctggtgcagtctggacctgaggtgaagaaccctggggcctcagtgaaggtctcctgcaaggcttctggttacacctttaccacctatggtatcagttgggtacgacaggcccctggacaagggcttgagtggatgggatggatcagcggttacaatggtaaaacaaacgatgcacagaagttccaggacagagtcgccatgaccacagacacatccacgagcacagcctacatggagctgaggagcctgagatctgacgacacggccatttattactgttcgagagatcgtttagtagtaccacctgccctttattattactactacgttatggacgtctggggccaagggaccacggtcaccgtctcctca

SEQ ID NO: 674 - protein, 127 aa, Artificial Sequence
  Synthetic
QVQLVQSGPEVKNPGASVKVSCKASGYTFTTYGISWVRQAPGQGLEWMGWISGYNGKTNDAQKFQDRVAMTTDTSTSTAYMELRSLRSDDTAIYYCSRDRLVVPPALYYYYYVMDVWGQGTTVTVSS

SEQ ID NO: 675 - DNA, 24 bp, Artificial Sequence
  Synthetic
ggttacacctttaccacctatggt

SEQ ID NO: 676 - protein, 8 aa, Artificial Sequence
  Synthetic
GYTFTTYG

SEQ ID NO: 677 - DNA, 24 bp, Artificial Sequence
  Synthetic
atcagcggttacaatggtaaaaca

SEQ ID NO: 678 - protein, 8 aa, Artificial Sequence
  Synthetic
ISGYNGKT

SEQ ID NO: 679 - DNA, 60 bp, Artificial Sequence
  Synthetic
tcgagagatcgtttagtagtaccacctgccctttattattactactacgttatggacgtc

SEQ ID NO: 680 - protein, 20 aa, Artificial Sequence
  Synthetic
SRDRLVVPPALYYYYYVMDV

SEQ ID NO: 681 - DNA, 336 bp, Artificial Sequence; identical to SEQ ID NO: 633
  Synthetic

SEQ ID NO: 682 - protein, 112 aa, Artificial Sequence; identical to SEQ ID NO: 336
  Synthetic

SEQ ID NO: 683 - DNA, 33 bp, Artificial Sequence; identical to SEQ ID NO: 323
  Synthetic

SEQ ID NO: 684 - protein, 11 aa, Artificial Sequence
  Synthetic
QSLVYSDGNTY

SEQ ID NO: 685 - DNA, 9 bp, Artificial Sequence
  Synthetic
aaggtttct

SEQ ID NO: 686 - protein, 3 aa, Artificial Sequence
  Synthetic
KVS

SEQ ID NO: 687 - DNA, 27 bp, Artificial Sequence
  Synthetic
atgcaaggtacacactggccgtacact

SEQ ID NO: 688 - protein, 9 aa, Artificial Sequence
  Synthetic
MQGTHWPYT

SEQ ID NO: 689 - DNA, 381 bp, Artificial Sequence; identical to SEQ ID NO: 673
  Synthetic

SEQ ID NO: 690 - protein, 127 aa, Artificial Sequence; identical to SEQ ID NO: 674
  Synthetic

SEQ ID NO: 691 - DNA, 336 bp, Artificial Sequence; identical to SEQ ID NO: 633
  Synthetic

SEQ ID NO: 692 - protein, 112 aa, Artificial Sequence; identical to SEQ ID NO: 336
  Synthetic

SEQ ID NO: 693 - DNA, 381 bp, Artificial Sequence
  Synthetic
caggttcagctggtgcagtctggagctgaggtgaagaagcctggggcctcagtgaaggtctcctgcaaggcttctggttacacctttaccacctatggtatcagctgggtgcgacaggcccctggacaagggcttgagtggatgggatggatcagcggttacaatggtaaaacaaactatgcacagaagctccagggcagagtcaccatgaccacagacacatccacgagcacagcctacatggagctgaggagcctgagatctgacgacacggccgtgtattactgttcgagagatcgtttagtagtaccacctgccctttattattactactacgttatggacgtctgggggcaagggaccacggtcaccgtctcctca

SEQ ID NO: 694 - protein, 127 aa, Artificial Sequence
  Synthetic
QVQLVQSGAEVKKPGASVKVSCKASGYTFTTYGISWVRQAPGQGLEWMGWISGYNGKTNYAQKLQGRVTMTTDTSTSTAYMELRSLRSDDTAVYYCSRDRLVVPPALYYYYYVMDVWGQGTTVTVSS

SEQ ID NO: 695 - DNA, 336 bp, Artificial Sequence; identical to SEQ ID NO: 335
  Synthetic

SEQ ID NO: 696 - protein, 112 aa, Artificial Sequence; identical to SEQ ID NO: 336
  Synthetic

SEQ ID NO: 697 - DNA, 384 bp, Artificial Sequence; identical to SEQ ID NO: 361
  Synthetic

SEQ ID NO: 698 - protein, 128 aa, Artificial Sequence; identical to SEQ ID NO: 362
  Synthetic

SEQ ID NO: 699 - DNA, 24 bp, Artificial Sequence
  Synthetic
ggattcaccttcagtgaccactac

SEQ ID NO: 700 - protein, 8 aa, Artificial Sequence
  Synthetic
GFTFSDHY

SEQ ID NO: 701 - DNA, 24 bp, Artificial Sequence
  Synthetic
attagtaatgatggtggtaccaaa

SEQ ID NO: 702 - protein, 8 aa, Artificial Sequence
  Synthetic
ISNDGGTK

SEQ ID NO: 703 - DNA, 63 bp, Artificial Sequence; identical to SEQ ID NO: 367
  Synthetic

SEQ ID NO: 704 - protein, 21 aa, Artificial Sequence
  Synthetic
ARDQGYIGYDSYYYYSYGMDV

SEQ ID NO: 705 - DNA, 321 bp, Artificial Sequence
  Synthetic
aaaattgtgttgacgcagtctccaggcaccctgcctttgtttccaggggaaagagccaccctctcctgtagggccagtcagagtgttaacaacaaattcttagcctggtaccagcagaaatctggccaggctcccaggctcctcatctatggtgcatccagcagggccactggcatcccagacaggttcagtggcagtgggtctgggaccgacttcactctcaccatcagcggactggagcctgaagattttgaagtgtattattgtcaagtatatggtaactcactcactttcggcggagggaccaaggtggagatcaag

SEQ ID NO: 706 - protein, 107 aa, Artificial Sequence
  Synthetic
KIVLTQSPGTLPLFPGERATLSCRASQSVNNKFLAWYQQKSGQAPRLLIYGASSRATGIPDRFSGSGSGTDFTLTISGLEPEDFEVYYCQVYGNSLTFGGGTKVEIK

SEQ ID NO: 707 - DNA, 21 bp, Artificial Sequence
  Synthetic
cagagtgttaacaacaaattc

SEQ ID NO: 708 - protein, 7 aa, Artificial Sequence
  Synthetic
QSVNNKF

SEQ ID NO: 709 - DNA, 9 bp, Artificial Sequence
  Synthetic
ggtgcatcc

SEQ ID NO: 710 - protein, 3 aa, Artificial Sequence
  Synthetic
GAS

SEQ ID NO: 711 - DNA, 24 bp, Artificial Sequence
  Synthetic
caagtatatggtaactcactcact

SEQ ID NO: 712 - protein, 8 aa, Artificial Sequence
  Synthetic
QVYGNSLT

SEQ ID NO: 713 - DNA, 384 bp, Artificial Sequence; identical to SEQ ID NO: 377
  Synthetic

SEQ ID NO: 714 - protein, 128 aa, Artificial Sequence; identical to SEQ ID NO: 378
  Synthetic

SEQ ID NO: 715 - DNA, 321 bp, Artificial Sequence
  Synthetic
gaaattgtgttgacgcagtctccaggcaccctgcctttgtttccaggggaaagagccaccctctcctgtagggccagtcagagtgttaacaacaaattcttagcctggtaccagcagaaatctggccaggctcccaggctcctcatctatggtgcatccagcagggccactggcatcccagacaggttcagtggcagtgggtctgggaccgacttcactctcaccatcagcggactggagcctgaagattttgaagtgtattattgtcaagtatatggtaactcactcactttcggcggagggaccaaggtggagatcaaa

SEQ ID NO: 716 - protein, 107 aa, Artificial Sequence
  Synthetic
EIVLTQSPGTLPLFPGERATLSCRASQSVNNKFLAWYQQKSGQAPRLLIYGASSRATGIPDRFSGSGSGTDFTLTISGLEPEDFEVYYCQVYGNSLTFGGGTKVEIK

SEQ ID NO: 717 - DNA, 384 bp, Artificial Sequence; identical to SEQ ID NO: 381
  Synthetic

SEQ ID NO: 718 - protein, 128 aa, Artificial Sequence; identical to SEQ ID NO: 382
  Synthetic

SEQ ID NO: 719 - DNA, 321 bp, Artificial Sequence; identical to SEQ ID NO: 383
  Synthetic

SEQ ID NO: 720 - protein, 107 aa, Artificial Sequence; identical to SEQ ID NO: 384
  Synthetic

SEQ ID NO: 721 - DNA, 378 bp, Artificial Sequence; identical to SEQ ID NO: 505
  Synthetic

SEQ ID NO: 722 - protein, 126 aa, Artificial Sequence; identical to SEQ ID NO: 506
  Synthetic

SEQ ID NO: 723 - DNA, 24 bp, Artificial Sequence
  Synthetic
ggttacacctttaccaactacgct

SEQ ID NO: 724 - protein, 8 aa, Artificial Sequence
  Synthetic
GYTFTNYA

SEQ ID NO: 725 - DNA, 24 bp, Artificial Sequence
  Synthetic
gtcagcgcttacaatggtcacaca

SEQ ID NO: 726 - protein, 8 aa, Artificial Sequence
  Synthetic
VSAYNGHT

SEQ ID NO: 727 - DNA, 57 bp, Artificial Sequence; identical to SEQ ID NO: 511
  Synthetic

SEQ ID NO: 728 - protein, 19 aa, Artificial Sequence
  Synthetic
ARGGVVVPVAPHFYNGMDV

SEQ ID NO: 729 - DNA, 336 bp, Artificial Sequence
  Synthetic
gatattgtgatgactcagtttccactctccctgcccgtcacccctggagagccggcctccatctcctgcaggtctagtcagagcctcctgcatattaatgaatacaactatttggattggtacctaaagaagccagggcagtctccacagctcctgatctatttgggttttaatcgggcctccggggtccctgacaggttcagtggcagtggatcaggcacagattttacactgaaaatcagcagagtggaggctgaggatgttggggtctattactgcatgcaagctcttcaaactccgtggacgttcggccaagggaccaaggtggaaatcaaa

SEQ ID NO: 730 - protein, 112 aa, Artificial Sequence
  Synthetic
DIVMTQFPLSLPVTPGEPASISCRSSQSLLHINEYNYLDWYLKKPGQSPQLLIYLGFNRASGVPDRFSGSGSGTDFTLKISRVEAEDVGVYYCMQALQTPWTFGQGTKVEIK

SEQ ID NO: 731 - DNA, 33 bp, Artificial Sequence; identical to SEQ ID NO: 515
  Synthetic

SEQ ID NO: 732 - protein, 11 aa, Artificial Sequence
  Synthetic
QSLLHINEYNY

SEQ ID NO: 733 - DNA, 9 bp, Artificial Sequence
  Synthetic
ttgggtttt

SEQ ID NO: 734 - protein, 3 aa, Artificial Sequence
  Synthetic
LGF

SEQ ID NO: 735 - DNA, 27 bp, Artificial Sequence
  Synthetic
atgcaagctcttcaaactccgtggacg

SEQ ID NO: 736 - protein, 9 aa, Artificial Sequence
  Synthetic
MQALQTPWT

SEQ ID NO: 737 - DNA, 378 bp, Artificial Sequence; identical to SEQ ID NO: 521
  Synthetic

SEQ ID NO: 738 - protein, 126 aa, Artificial Sequence; identical to SEQ ID NO: 522
  Synthetic

SEQ ID NO: 739 - DNA, 336 bp, Artificial Sequence
  Synthetic
gatattgtgatgactcagtctccactctccctgcccgtcacccctggagagccggcctccatctcctgcaggtctagtcagagcctcctgcatattaatgaatacaactatttggattggtacctaaagaagccagggcagtctccacagctcctgatctatttgggttttaatcgggcctccggggtccctgacaggttcagtggcagtggatcaggcacagattttacactgaaaatcagcagagtggaggctgaggatgttggggtctattactgcatgcaagctcttcaaactccgtggacgttcggccaagggaccaaggtggaaatcaaa

SEQ ID NO: 740 - protein, 112 aa, Artificial Sequence
  Synthetic
DIVMTQSPLSLPVTPGEPASISCRSSQSLLHINEYNYLDWYLKKPGQSPQLLIYLGFNRASGVPDRFSGSGSGTDFTLKISRVEAEDVGVYYCMQALQTPWTFGQGTKVEIK

SEQ ID NO: 741 - DNA, 378 bp, Artificial Sequence; identical to SEQ ID NO: 525
  Synthetic

SEQ ID NO: 742 - protein, 126 aa, Artificial Sequence; identical to SEQ ID NO: 526
  Synthetic

SEQ ID NO: 743 - DNA, 336 bp, Artificial Sequence; identical to SEQ ID NO: 527
  Synthetic

SEQ ID NO: 744 - protein, 112 aa, Artificial Sequence; identical to SEQ ID NO: 528
  Synthetic

SEQ ID NO: 745 - protein, 8 aa, Artificial Sequence
  Synthetic
  VARIANT (1)...(8): Xaa = Any amino acid
XXXXXXXX

SEQ ID NO: 746 - protein, 8 aa, Artificial Sequence
  Synthetic
  VARIANT (1)...(8): Xaa - Any amino acid
XXXXXXXX

SEQ ID NO: 747 - protein, 20 aa, Artificial Sequence
  Synthetic
  VARIANT (1)...(20): Xaa = Any amino acid
XXXXXXXXXXXXXXXXXXXX

SEQ ID NO: 748 - protein, 12 aa, Artificial Sequence
  Synthetic
  VARIANT (1)...(12): Xaa = Any amino acid
XXXXXXXXXXXX

SEQ ID NO: 749 - protein, 3 aa, Artificial Sequence
  Synthetic
  VARIANT (1)...(3): Xaa = Any amino acid
XXX

SEQ ID NO: 750 - protein, 9 aa, Artificial Sequence
  Synthetic
  VARIANT (1)...(9): Xaa = Any amino acid
XXXXXXXXX

SEQ ID NO: 751 - protein, 330 aa, Artificial Sequence [sequence omitted]

SEQ ID NO: 752 - protein, 327 aa, Artificial Sequence
  Synthetic
ASTKGPSVFPLAPCSRSTSESTAALGCLVKDYFPEPVTVSWNSGALTSGVHTFPAVLQSSGLYSLSSVVTVPSSSLGTKTYTCNVDHKPSNTKVDKRVESKYGPPCPSCPAPEFLGGPSVFLFPPKPKDTLMISRTPEVTCVVVDVSQEDPEVQFNWYVDGVEVHNAKTKPREEQFNSTYRVVSVLTVLHQDWLNGKEYKCKVSNKGLPSSIEKTISKAKGQPREPQVYTLPPSQEEMTKNQVSLTCLVKGFYPSDIAVEWESNGQPENNYKTTPPVLDSDGSFFLYSRLTVDKSRWQEGNVFSCSVMHEALHNHYTQKSLSLSLGK

SEQ ID NO: 753 - protein, 327 aa, Artificial Sequence
  Synthetic
ASTKGPSVFPLAPCSRSTSESTAALGCLVKDYFPEPVTVSWNSGALTSGVHTFPAVLQSSGLYSLSSVVTVPSSSLGTKTYTCNVDHKPSNTKVDKRVESKYGPPCPPCPAPEFLGGPSVFLFPPKPKDTLMISRTPEVTCVVVDVSQEDPEVQFNWYVDGVEVHNAKTKPREEQFNSTYRVVSVLTVLHQDWLNGKEYKCKVSNKGLPSSIEKTISKAKGQPREPQVYTLPPSQEEMTKNQVSLTCLVKGFYPSDIAVEWESNGQPENNYKTTPPVLDSDGSFFLYSRLTVDKSRWQEGNVFSCSVMHEALHNHYTQKSLSLSLGK

SEQ ID NO: 754 - DNA, 2076 bp, Homo sapiens
atgggcaccgtcagctccaggcggtcctggtggccgctgccactgctgctgctgctgctgctgctcctgggtcccgcgggcgcccgtgcgcaggaggacgaggacggcgactacgaggagctggtgctagccttgcgttccgaggaggacggcctggccgaagcacccgagcacggaaccacagccaccttccaccgctgcgccaaggatccgtggaggttgcctggcacctacgtggtggtgctgaaggaggagacccacctctcgcagtcagagcgcactgcccgccgcctgcaggcccaggctgcccgccggggatacctcaccaagatcctgcatgtcttccatggccttcttcctggcttcctggtgaagatgagtggcgacctgctggagctggccttgaagttgccccatgtcgactacatcgaggaggactcctctgtctttgcccagagcatcccgtggaacctggagcggattacccctccacggtaccgggcggatgaataccagccccccgacggaggcagcctggtggaggtgtatctcctagacaccagcatacagagtgaccaccgggaaatcgagggcagggtcatggtcaccgacttcgagaatgtgcccgaggaggacgggacccgcttccacagacaggccagcaagtgtgacagtcatggcacccacctggcaggggtggtcagcggccgggatgccggcgtggccaagggtgccagcatgcgcagcctgcgcgtgctcaactgccaagggaagggcacggttagcggcaccctcataggcctggagtttattcggaaaagccagctggtccagcctgtggggccactggtggtgctgctgcccctggcgggtgggtacagccgcgtcctcaacgccgcctgccagcgcctggcgagggctggggtcgtgctggtcaccgctgccggcaacttccgggacgatgcctgcctctactccccagcctcagctcccgaggtcatcacagttggggccaccaatgcccaggaccagccggtgaccctggggactttggggaccaactttggccgctgtgtggacctctttgccccaggggaggacatcattggtgcctccagcgactgcagcacctgctttgtgtcacagagtgggacatcacaggctgctgcccacgtggctggcattgcagccatgatgctgtctgccgagccggagctcaccctggccgagttgaggcagagactgatccacttctctgccaaagatgtcatcaatgaggcctggttccctgaggaccagcgggtactgacccccaacctggtggccgccctgccccccagcacccatggggcaggttggcagctgttttgcaggactgtgtggtcagcacactcggggcctacacggatggccacagccatcgcccgctgcgccccagatgaggagctgctgagctgctccagtttctccaggagtgggaagcggcggggcgagcgcatggaggcccaagggggcaagctggtctgccgggcccacaacgcttttgggggtgagggtgtctacgccattgccaggtgctgcctgctaccccaggccaactgcagcgtccacacagctccaccagctgaggccagcatggggacccgtgtccactgccaccaacagggccacgtcctcacaggctgcagctcccactgggaggtggaggaccttggcacccacaagccgcctgtgctgaggccacgaggtcagcccaaccagtgcgtgggccacagggaggccagcatccacgcttcctgctgccatgccccaggtctggaatgcaaagtcaaggagcatggaatcccggcccctcaggagcaggtgaccgtggcctgcgaggagggctggaccctgactggctgcagtgccctccctgggacctcccacgtcctgggggcctacgccgtagacaacacgtgtgtagtcaggagccgggacgtcagcactacaggcagcaccagcgaagaggccgtgacagccgttgccatctgctgccggagccggcacctggcgcaggcctcccaggagctccag

SEQ ID NO: 755 - protein, 692 aa, Homo sapiens
MGTVSSRRSWWPLPLLLLLLLLLGPAGARAQEDEDGDYEELVLALRSEEDGLAEAPEHGTTATFHRCAKDPWRLPGTYVVVLKEETHLSQSERTARRLQAQAARRGYLTKILHVFHGLLPGFLVKMSGDLLELALKLPHVDYIEEDSSVFAQSIPWNLERITPPRYRADEYQPPDGGSLVEVYLLDTSIQSDHREIEGRVMVTDFENVPEEDGTRFHRQASKCDSHGTHLAGVVSGRDAGVAKGASMRSLRVLNCQGKGTVSGTLIGLEFIRKSQLVQPVGPLVVLLPLAGGYSRVLNAACQRLARAGVVLVTAAGNFRDDACLYSPASAPEVITVGATNAQDQPVTLGTLGTNFGRCVDLFAPGEDIIGASSDCSTCFVSQSGTSQAAAHVAGIAAMMLSAEPELTLAELRQRLIHFSAKDVINEAWFPEDQRVLTPNLVAALPPSTHGAGWQLFCRTVWSAHSGPTRMATAIARCAPDEELLSCSSFSRSGKRRGERMEAQGGKLVCRAHNAFGGEGVYAIARCCLLPQANCSVHTAPPAEASMGTRVHCHQQGHVLTGCSSHWEVEDLGTHKPPVLRPRGQPNQCVGHREASIHASCCHAPGLECKVKEHGIPAPQEQVTVACEEGWTLTGCSALPGTSHVLGAYAVDNTCVVRSRDVSTTGSTSEEAVTAVAICCRSRHLAQASQELQ

SEQ ID NO: 756 - protein, 692 aa, Macaca mulata
MGTVSSRRSWWPLPLPLLLLLLLGPAGARAQEDEDGDYEELVLALRSEEDGLADAPEHGATATFHRCAKDPWRLPGTYVVVLKEETHRSQSERTARRLQAQAARRGYLTKILHVFHHLLPGFLVKMSGDLLELALKLPHVDYIEEDSSVFAQSIPWNLERITPARYRADEYQPPKGGSLVEVYLLDTSIQSDHREIEGRVMVTDFESVPEEDGTRFHRQASKCDSHGTHLAGVVSGRDAGVAKGAGLRSLRVLNCQGKGTVSGTLIGLEFIRKSQLVQPVGPLVVLLPLAGGYSRVFNAACQRLARAGVVLVTAAGNFRDDACLYSPASAPEVITVGATNAQDQPVTLGTLGTNFGRCVDLFAPGEDIIGASSDCSTCFVSRSGTSQAAAHVAGIAAMMLSAEPELTLAELRQRLIHFSAKDVINEAWFPEDQRVLTPNLVAALPPSTHRAGWQLFCRTVWSAHSGPTRMATAVARCAQDEELLSCSSFSRSGKRRGERIEAQGGKRVCRAHNAFGGEGVYAIARCCLLPQVNCSVHTAPPAGASMGTRVHCHQQGHVLTGCSSHWEVEDLGTHKPPVLRPRGQPNQCVGHREASIHASCCHAPGLECKVKEHGIPAPQEQVIVACEDGWTLTGCSPLPGTSHVLGAYAVDNTCVVRSRDVSTTGSTSKEAVAAVAICCRSRHLVQASQELQ

SEQ ID NO: 757 - protein, 694 aa, Mus muscular
MGTHCSAWLRWPLLPLLPPLLLLLLLLCPTGAGAQDEDGDYEELMLALPSQEDGLADEAAHVATATFRRCSKEAWRLPGTYIVVLMEETQRLQIEQTAHRLQTRAARRGYVIKVLHIFYDLFPGFLVKMSSDLLGLALKLPHVEYIEEDSFVFAQSIPWNLERIIPAWHQTEEDRSPDGSSQVEVYLLDTSIQGAHREIEGRVTITDFNSVPEEDGTRFHRQASKCDSHGTHLAGVVSGRDAGVAKGTSLHSLRVLNCQGKGTVSGTLIGLEFIRKSQLIQPSGPLVVLLPLAGGYSRILNAACRHLARTGVVLVAAAGNFRDDACLYSPASAPEVITVGATNAQDQPVTLGTLGTNFGRCVDLFAPGKDIIGASSDCSTCFMSQSGTSQAAAHVAGIVARMLSREPTLTLAELRQRLIHFSTKDVINMAWFPEDQQVLTPNLVATLPPSTHETGGQLLCRTVWSAHSGPTRTATATARCAPEEELLSCSSFSRSGRRRGDWIEAIGGQQVCKALNAFGGEGVYAVARCCLVPRANCSIHNTPAARAGLETHVHCHQKDHVLTGCSFHWEVEDLSVRRQPALRSRRQPGQCVGHQAASVYASCCHAPGLECKIKEHGISGPSEQVTVACEAGWTLTGCNVLPGASLTLGAYSVDNLCVARVHDTARADRTSGEATVAAAICCRSRPSAKASWVQ

SEQ ID NO: 758 - protein, 653 aa, Homo sapiens
EFRCHDGKCISRQFVCDSDRDCLDGSDEASCPVLTCGPASFQCNSSTCIPQLWACDNDPDCEDGSDEWPQRCRGLYVFQGDSSPCSAFEFHCLSGECIHSSWRCDGGPDCKDKSDEENCAVATCRPDEFQCSDGNCIHGSRQCDREYDCKDMSDEVGCVNVTLCEGPNKFKCHSGECITLDKVCNMARDCRDWSDEPIKECGTNECLDNNGGCSHVCNDLKIGYECLCPDGFQLVAQRRCEDIDECQDPDTCSQLCVNLEGGYKCQCEEGFQLDPHTKACKAVGSIAYLFFTNRHEVRKMTLDRSEYTSLIPNLRNVVALDTEVASNRIYWSDLSQRMICSTQLDRAHGVSSYDTVISRDIQAPDGLAVDWIHSNIYWTDSVLGTVSVADTKGVKRKTLFRENGSKPRAIVVDPVHGFMYWTDWGTPAKIKKGGLNGVDIYSLVTENIQWPNGITLDLLSGRLYWVDSKLHSISSIDVNGGNRKTILEDEKRLAHPFSLAVFEDKVFWTDIINEAIFSANRLTGSDVNLLAENLLSPEDMVLFHNLTQPRGVNWCERTTLSNGGCQYLCLPAPQINPHSPKFTCACPDGMLLARDMRSCLTEAEAAVATQETSTVRLKVSSTAVRTQHTTTRPVPDTSRLPGATPGLTTVEIV

SEQ ID NO: 759 - protein, 753 aa, Homo sapiens
MERRAWSLQCTAFVLFCAWCALNSAKAKRQFVNEWAAEIPGGPEAASAIAEELGYDLLGQIGSLENHYLFKHKNHPRRSRRSAFHITKRLSDDDRVIWAEQQYEKERSKRSALRDSALNLFNDPMWNQQWYLQDTRMTAALPKLDLHVIPVWQKGITGKGVVITVLDDGLEWNHTDIYANYDPEASYDFNDNDHDPFPRYDPTNENKHGTRCAGEIAMQANNHKCGVGVAYNSKVGGIRMLDGIVTDAIEASSIGFNPGHVDIYSASWGPNDDGKTVEGPGRLAQKAFEYGVKQGRQGKGSIFVWASGNGGRQGDNCDCDGYTDSIYTISISSASQQGLSPWYAEKCSSTLATSYSSGDYTDQRITSADLHNDCTETHTGTSASAPLAAGIFALALEANPNLTWRDMQHLVVWTSEYDPLANNPGWKKNGAGLMVNSRFGFGLLNAKALVDLADPRTWRSVPEKKECVVKDNDFEPRALKANGEVIIEIPTRACEGQENAIKSLEHVQFEATIEYSRRGDLHVTLTSAAGTSTVLLAERERDTSPNGFKNWDFMSVHTWGENPIGTWTLRITDMSGRIQNEGRIVNWKLILHGTSSQPEHMKQPRVYTSYNTVQNDRRGVEKMVDPGEEQPTQENPKENTLVSKSPSSSSVGGRRDELEEGAPSQAMLRLLQSAFSKNSPPKQSPKKSPSAKLNIPYENFYEALEKLNKPSQLKDSEDSLYNDYVDVFYNTKPYKHRDDRLLQALVDILNEEN

SEQ ID NO: 760 - protein, 785 aa, Homo sapiens
MPKGRQKVPHLDAPLGLPTCLWLELAGLFLLVPWVMGLAGTGGPDGQGTGGPSWAVHLESLEGDGEEETLEQQADALAQAAGLVNAGRIGELQGHYLFVQPAGHRPALEVEAIRQQVEAVLAGHEAVRWHSEQRLLRRAKRSVHFNDPKYPQQWHLNNRRSPGRDINVTGVWERNVTGRGVTVVVVDDGVEHTIQDIAPNYSPEGSYDLNSNDPDPMPHPDVENGNHHGTRCAGEIAAVPNNSFCAVGVAYGSRIAGIRVLDGPLTDSMEAVAFNKHYQINDIYSCSWGPDDDGKTVDGPHQLGKAALQHGVIAGRQGFGSIFVVASGNGGQHNDNCNYDGYANSIYTVTIGAVDEEGRMPFYAEECASMLAVTFSGGDKMLRSIVTTDWDLQKGTGCTEGHTGTSAAAPLAAGMIALMLQVRPCLTWRDVQHIIVFTATRYEDRRAEWVTNEAGFSHSHQHGFGLLNAWRLVNAAKIWTSVPYLASYVSPVLKENKAIPQSPRSLEVLWNVSRMDLEMSGLKTLEHVAVTVSITHPRRGSLELKLFCPSGMMSLIGAPRSMDSDPNGFNDWTFSTVRCWGERARGTYRLVIRDVGDESFQVGILRQWQLTLYGSVWSAVDIRDRQRLLESAMSGKYLHDDFALPCPPGLKIPEEDGYTITPNTLKTLVLVGCFTVFWTVYYMLEVYLSQRNVASNQVCRSGPCHWPHRSRKAKEEGTELESVPLCSSKDPDEVETESRGPPTTSDLLAPDLLEQGDWSLSQNKSALDCPHQHLDVPHGKEEQIC

SEQ ID NO: 761 - protein, 692 aa, Macaca fascicularis
MGTVSSRRSWWPLPLPLLLLLLLGPAGARAQEDEDGDYEELVLALRSEEDGLADAPEHGATATFHRCAKDPWRLPGTYVVVLKEETHRSQSERTARRLQAQAARRGYLTKILHVFHHLLPGFLVKMSGDLLELALKLPHVDYIEEDSSVFAQSIPWNLERITPARYRADEYQPPKGGSLVEVYLLDTSIQSDHREIEGRVMVTDFESVPEEDGTRFHRQASKCDSHGTHLAGVVSGRDAGVAKGAGLRSLRVLNCQGKGTVSGTLIGLEFIRKSQLVQPVGPLVVLLPLAGGYSRVFNAACQRLARAGVVLVTAAGNFRDDACLYSPASAPEVITVGATNAQDQPVTLGTLGTNFGRCVDLFAPGEDIIGASSDCSTCFVSRSGTSQAAAHVAGIAAMMLSAEPELTLAELRQRLIHFSAKDVINEAWFPEDQRVLTPNLVAALPPSTHRAGWQLFCRTVWSAHSGPTRMATAVARCAQDEELLSCSSFSRSGKRRGERIEAQGGKRVCRAHNAFGGEGVYAIARCCLLPQVNCSVHTAPPAGASMGTRVHCHQQGHVLTGCSSHWEVEDLGTHKPPVLRPRGQPNQCVGHREASIHASCCHAPGLECKVKEHGIPAPQEQVIVACEDGWTLTGCSALPGTSHVLGAYAVDNTCVVRSRDVSTTGSTSEEAVAAVAICCRSRHLVQASQELQ

SEQ ID NO: 762 - protein, 698 aa, Mesocricetus auratus
MGTSCSARPRWLLSPLLLLLLLLRYMGASAQDEDAEYEELMLTLQSQDDGLADETDEAPQGATAAFHRCPEEAWRVPGTYIVMLAEEAQWVHIEQTMHRLQTQAARRGYVIKIQHIFYDFLPAFVVKMSSDLLDLALKLPHVKYIEEDSLVFAQSIPWNLDRIIPAGRQAQEYSSSRKVPSGSGQVEVYLLDTSIQSDHREIEGRVTVTDFNSVPEEDGTRFHRQASKCDSHGTHLAGVVSGRDAGVAKGTILHGLRVLNCQGKGIVSGILTGLEFIWKSQLMQPSGPQVVLLPLAGRYSRVLNTACQHLARTGVVLVAAAGNFRDDACLYSPASAPEVITVGATDVQDQPVTLGTLGTNFGRCVDLFAPGKDIIGASSDCSACFMSQSGTSQAAAHVAGIVAMMLTLEPELTLTELRQRLIHFSTKDAINMAWFPEDQRVLTPNLVATLPPSTHGTGGQLLCRTVWSAHSGPTRAATATARCAPGEELLSCSSFSRSGRRRGDRIEAAGTQQVCKALNAFGGEGVYAVARCCLLPRANCSIHTTPAARTSLETHAHCHQKDHVLTGCSLHWEVEGIGVQPLAVLRSRHQPGQCTGHREASVHASCCHAPGLECKIKEHGISGPAEQVTVACEAGWTLTGCNVLPGAFITLGAYAVDNTCVARSRVTDTAGRTGEEATVAAAICCRNRPSAKASWVHQ

SEQ ID NO: 763 - protein, 691 aa, Rattus norvegicus
MGIRCSTWLRWPLSPQLLLLLLLCPTGSRAQDEDGDYEELMLALPSQEDSLVDEASHVATATFRRCSKEAWRLPGTYVVVLMEETQRLQVEQTAHRLQTWAARRGYVIKVLHVFYDLFPGFLVKMSSDLLGLALKLPHVEYIEEDSLVFAQSIPWNLERIIPAWQQTEEDSSPDGSSQVEVYLLDTSIQSGHREIEGRVTITDFNSVPEEDGTRFHRQASKCDSHGTHLAGVVSGRDAGVAKGTSLHSLRVLNCQGKGTVSGTLIGLEFIRKSQLIQPSGPLVVLLPLAGGYSRILNTACQRLARTGVVLVAAAGNFRDDACLYSPASAPEVITVGATNAQDQPVTLGTLGTNFGRCVDLFAPGKDIIGASSDCSTCYMSQSGTSQAAAHVAGIVAMMLNRDPALTLAELRQRLILFSTKDVINMAWFPEDQRVLTPNRVATLPPSTQETGGQLLCRTVWSAHSGPTRTATATARCAPEEELLSCSSFSRSGRRRGDRIEAIGGQQVCKALNAFGGEGVYAVARCCLLPRVNCSIHNTPAARAGPQTPVHCHQKDHVLTGCSFHWEVENLRAQQQPLLRSRHQPGQCVGHQEASVHASCCHAPGLECKIKEHGIAGPAEQVTVACEAGWTLTGCNVLPGASLPLGAYSVDNVCVARIRDAGRADRTSEEATVAAAICCRSRPSAKASWVHQ